European Patent Specification EP 3 055 676 B1, published July 8, 2026. Title: METHODS AND SYSTEMS FOR DIGITALLY COUNTING FEATURES ON ARRAYS. Applicant: FU, GLENN RUDOFF, ROGER STERN, DAVID WU, GEORGE T. FODOR, STEPHEN P.A. FACER, GEOFF. Application US 14/508,911. The sequence listing filed with the application follows.

SEQUENCE LISTING (961 sequences)

SEQ ID NO: 1 - DNA, 25 bp, Artificial Sequence
  Description of Artificial Sequence: Synthetic probe
  5' amino modifier C6
tcctgaacggtagcatcttgacgac

SEQ ID NO: 2 - DNA, 28 bp, Artificial Sequence
  Description of Artificial Sequence: Synthetic probe
  5' amino modifier C6
cccaaagggtaccagagcttaaggtcaa

SEQ ID NO: 3 - DNA, 28 bp, Artificial Sequence
  Description of Artificial Sequence: Synthetic probe
  5' amino modifier C6
cccaaagcgttaaggtttcttgtcacaa

SEQ ID NO: 4 - DNA, 28 bp, Artificial Sequence
  Description of Artificial Sequence: Synthetic probe
  5' amino modifier C6
cccaagtcgtacgaactcaccacatgaa

SEQ ID NO: 5 - DNA, 28 bp, Artificial Sequence
  Description of Artificial Sequence: Synthetic probe
  5' amino modifier C6
cccaaacttgttcccttgagaccagtaa

SEQ ID NO: 6 - DNA, 28 bp, Artificial Sequence
  Description of Artificial Sequence: Synthetic probe
  5' amino modifier C6
cccaagacttctaccctaggttccagaa

SEQ ID NO: 7 - DNA, 28 bp, Artificial Sequence
  Description of Artificial Sequence: Synthetic probe
  5' amino modifier C6
cccaaccagacttgggtacgtgaaacaa

SEQ ID NO: 8 - DNA, 28 bp, Artificial Sequence
  Description of Artificial Sequence: Synthetic probe
  5' amino modifier C6
cccaacgactggttctgaagtggaacaa

SEQ ID NO: 9 - DNA, 28 bp, Artificial Sequence
  Description of Artificial Sequence: Synthetic probe
  5' amino modifier C6
cccaatttagcttcgtgagtcagaccaa

SEQ ID NO: 10 - DNA, 28 bp, Artificial Sequence
  Description of Artificial Sequence: Synthetic probe
  5' amino modifier C6
cccaactcgaagagtggtcagtctttaa

SEQ ID NO: 11 - DNA, 28 bp, Artificial Sequence
  Description of Artificial Sequence: Synthetic probe
  5' amino modifier C6
cccaatcgcaaggagacatagtctttaa

SEQ ID NO: 12 - DNA, 28 bp, Artificial Sequence
  Description of Artificial Sequence: Synthetic probe
  5' amino modifier C6
cccaagtcctagtgagagcaacgtttaa

SEQ ID NO: 13 - DNA, 28 bp, Artificial Sequence
  Description of Artificial Sequence: Synthetic probe
  5' amino modifier C6
cccaaggaacctactgtccttgtcagaa

SEQ ID NO: 14 - DNA, 28 bp, Artificial Sequence
  Description of Artificial Sequence: Synthetic probe
  5' amino modifier C6
cccaaactagaagacgagttcgagtcaa

SEQ ID NO: 15 - DNA, 28 bp, Artificial Sequence
  Description of Artificial Sequence: Synthetic probe
  5' amino modifier C6
cccaaggacatactcaacgtagctcaaa

SEQ ID NO: 16 - DNA, 28 bp, Artificial Sequence
  Description of Artificial Sequence: Synthetic probe
  5' amino modifier C6
cccaaggcatttgcaacctcacatgaaa

SEQ ID NO: 17 - DNA, 28 bp, Artificial Sequence
  Description of Artificial Sequence: Synthetic probe
  5' amino modifier C6
cccaagtacccatccactgtcgagtaaa

SEQ ID NO: 18 - DNA, 28 bp, Artificial Sequence
  Description of Artificial Sequence: Synthetic probe
  5' amino modifier C6
cccaaagcgtttgtgtaacagaccataa

SEQ ID NO: 19 - DNA, 28 bp, Artificial Sequence
  Description of Artificial Sequence: Synthetic probe
  5' amino modifier C6
cccaaatggtctggttcgacagtcacaa

SEQ ID NO: 20 - DNA, 28 bp, Artificial Sequence
  Description of Artificial Sequence: Synthetic probe
  5' amino modifier C6
cccaagaggtacaacgactctagggtaa

SEQ ID NO: 21 - DNA, 28 bp, Artificial Sequence
  Description of Artificial Sequence: Synthetic probe
  5' amino modifier C6
cccaagaacttctacttgcttcgtgaaa

SEQ ID NO: 22 - DNA, 28 bp, Artificial Sequence
  Description of Artificial Sequence: Synthetic probe
  5' amino modifier C6
cccaagcactttctgttaactagctgaa

SEQ ID NO: 23 - DNA, 28 bp, Artificial Sequence
  Description of Artificial Sequence: Synthetic probe
  5' amino modifier C6
cccaagaacctctctctagtgctagtaa

SEQ ID NO: 24 - DNA, 28 bp, Artificial Sequence
  Description of Artificial Sequence: Synthetic probe
  5' amino modifier C6
cccaagcctttaagcctaaagtcctgaa

SEQ ID NO: 25 - DNA, 28 bp, Artificial Sequence
  Description of Artificial Sequence: Synthetic probe
  5' amino modifier C6
cccaatctggtagctcaacatccttgaa

SEQ ID NO: 26 - DNA, 28 bp, Artificial Sequence
  Description of Artificial Sequence: Synthetic probe
  5' amino modifier C6
cccaaaggactccatggagaagtgtcaa

SEQ ID NO: 27 - DNA, 28 bp, Artificial Sequence
  Description of Artificial Sequence: Synthetic probe
  5' amino modifier C6
cccaagaaccctttctggaagcttccaa

SEQ ID NO: 28 - DNA, 28 bp, Artificial Sequence
  Description of Artificial Sequence: Synthetic probe
  5' amino modifier C6
cccaaattcgcttcctagtagtggacaa

SEQ ID NO: 29 - DNA, 28 bp, Artificial Sequence
  Description of Artificial Sequence: Synthetic probe
  5' amino modifier C6
cccaaccgtacgaagacctagtttctaa

SEQ ID NO: 30 - DNA, 28 bp, Artificial Sequence
  Description of Artificial Sequence: Synthetic probe
  5' amino modifier C6
cccaatcacgaagagagtcactgtttaa

SEQ ID NO: 31 - DNA, 28 bp, Artificial Sequence
  Description of Artificial Sequence: Synthetic probe
  5' amino modifier C6
cccaagaaacataaactcgagttgcgaa

SEQ ID NO: 32 - DNA, 28 bp, Artificial Sequence
  Description of Artificial Sequence: Synthetic probe
  5' amino modifier C6
cccaaccagttacgtgagtgttgctaaa

SEQ ID NO: 33 - DNA, 28 bp, Artificial Sequence
  Description of Artificial Sequence: Synthetic probe
  5' amino modifier C6
cccaaactcgtgactcctgtttcagaaa

SEQ ID NO: 34 - DNA, 28 bp, Artificial Sequence
  Description of Artificial Sequence: Synthetic probe
  5' amino modifier C6
cccaacggttgaagagactcctgaaaaa

SEQ ID NO: 35 - DNA, 28 bp, Artificial Sequence
  Description of Artificial Sequence: Synthetic probe
  5' amino modifier C6
cccaaattgctctggtcacatcgaaaaa

SEQ ID NO: 36 - DNA, 28 bp, Artificial Sequence
  Description of Artificial Sequence: Synthetic probe
  5' amino modifier C6
cccaacaggacttgtgctacgtgttaaa

SEQ ID NO: 37 - DNA, 28 bp, Artificial Sequence
  Description of Artificial Sequence: Synthetic probe
  5' amino modifier C6
cccaaatttcgtgtgtcaaccatgccaa

SEQ ID NO: 38 - DNA, 28 bp, Artificial Sequence
  Description of Artificial Sequence: Synthetic probe
  5' amino modifier C6
cccaacgtgaaggcttaacaacattgaa

SEQ ID NO: 39 - DNA, 28 bp, Artificial Sequence
  Description of Artificial Sequence: Synthetic probe
  5' amino modifier C6
cccaatgaacacaactacgaagctgtaa

SEQ ID NO: 40 - DNA, 28 bp, Artificial Sequence
  Description of Artificial Sequence: Synthetic probe
  5' amino modifier C6
cccaaacttccgttgttactagtcgaaa

SEQ ID NO: 41 - DNA, 28 bp, Artificial Sequence
  Description of Artificial Sequence: Synthetic probe
  5' amino modifier C6
cccaaggagtacaagcttcctagggtaa

SEQ ID NO: 42 - DNA, 28 bp, Artificial Sequence
  Description of Artificial Sequence: Synthetic probe
  5' amino modifier C6
cccaagtgctaaactgctctttacgtaa

SEQ ID NO: 43 - DNA, 28 bp, Artificial Sequence
  Description of Artificial Sequence: Synthetic probe
  5' amino modifier C6
cccaaagaaactgcatctcctttggaaa

SEQ ID NO: 44 - DNA, 28 bp, Artificial Sequence
  Description of Artificial Sequence: Synthetic probe
  5' amino modifier C6
cccaaggactaagttccactcacctgaa

SEQ ID NO: 45 - DNA, 28 bp, Artificial Sequence
  Description of Artificial Sequence: Synthetic probe
  5' amino modifier C6
cccaaagttgtctggttcactcgagaaa

SEQ ID NO: 46 - DNA, 28 bp, Artificial Sequence
  Description of Artificial Sequence: Synthetic probe
  5' amino modifier C6
cccaacgttctaagtttgcttcgaagaa

SEQ ID NO: 47 - DNA, 28 bp, Artificial Sequence
  Description of Artificial Sequence: Synthetic probe
  5' amino modifier C6
cccaactaaaggttgtgcatccaagcaa

SEQ ID NO: 48 - DNA, 28 bp, Artificial Sequence
  Description of Artificial Sequence: Synthetic probe
  5' amino modifier C6
cccaaaggcttcacgacatgtcatttaa

SEQ ID NO: 49 - DNA, 28 bp, Artificial Sequence
  Description of Artificial Sequence: Synthetic probe
  5' amino modifier C6
cccaactgctaggttcctacacaagtaa

SEQ ID NO: 50 - DNA, 28 bp, Artificial Sequence
  Description of Artificial Sequence: Synthetic probe
  5' amino modifier C6
cccaaatcagtagctacaccacaggtaa

SEQ ID NO: 51 - DNA, 28 bp, Artificial Sequence
  Description of Artificial Sequence: Synthetic probe
  5' amino modifier C6
cccaagactgcaagctcactacattgaa

SEQ ID NO: 52 - DNA, 28 bp, Artificial Sequence
  Description of Artificial Sequence: Synthetic probe
  5' amino modifier C6
cccaagctactcctctaagagcatagaa

SEQ ID NO: 53 - DNA, 28 bp, Artificial Sequence
  Description of Artificial Sequence: Synthetic probe
  5' amino modifier C6
cccaatggaacgctaaggtgtaaaccaa

SEQ ID NO: 54 - DNA, 28 bp, Artificial Sequence
  Description of Artificial Sequence: Synthetic probe
  5' amino modifier C6
cccaagaaactaaccttggcttgccaaa

SEQ ID NO: 55 - DNA, 28 bp, Artificial Sequence
  Description of Artificial Sequence: Synthetic probe
  5' amino modifier C6
cccaaccattagaccttgtgttgccaaa

SEQ ID NO: 56 - DNA, 28 bp, Artificial Sequence
  Description of Artificial Sequence: Synthetic probe
  5' amino modifier C6
cccaaggtctgacagtaggtgttccaaa

SEQ ID NO: 57 - DNA, 28 bp, Artificial Sequence
  Description of Artificial Sequence: Synthetic probe
  5' amino modifier C6
cccaatttcgcaagccttggtacataaa

SEQ ID NO: 58 - DNA, 28 bp, Artificial Sequence
  Description of Artificial Sequence: Synthetic probe
  5' amino modifier C6
cccaagtttctagcctaccactacggaa

SEQ ID NO: 59 - DNA, 28 bp, Artificial Sequence
  Description of Artificial Sequence: Synthetic probe
  5' amino modifier C6
cccaaatagacctaacggaagctgtgaa

SEQ ID NO: 60 - DNA, 28 bp, Artificial Sequence
  Description of Artificial Sequence: Synthetic probe
  5' amino modifier C6
cccaaggagtcatccatgcatctttgaa

SEQ ID NO: 61 - DNA, 28 bp, Artificial Sequence
  Description of Artificial Sequence: Synthetic probe
  5' amino modifier C6
cccaaccgtactagcttgggttaaacaa

SEQ ID NO: 62 - DNA, 28 bp, Artificial Sequence
  Description of Artificial Sequence: Synthetic probe
  5' amino modifier C6
cccaaaaaggctagccttctgactttaa

SEQ ID NO: 63 - DNA, 28 bp, Artificial Sequence
  Description of Artificial Sequence: Synthetic probe
  5' amino modifier C6
cccaaagagctctgcactacaagtttaa

SEQ ID NO: 64 - DNA, 28 bp, Artificial Sequence
  Description of Artificial Sequence: Synthetic probe
  5' amino modifier C6
cccaacagctaacggtagtaaaggtcaa

SEQ ID NO: 65 - DNA, 28 bp, Artificial Sequence
  Description of Artificial Sequence: Synthetic probe
  5' amino modifier C6
cccaaagctttccgtttcaaagtgacaa

SEQ ID NO: 66 - DNA, 28 bp, Artificial Sequence
  Description of Artificial Sequence: Synthetic probe
  5' amino modifier C6
cccaagtccatgcttccagtgacaaaaa

SEQ ID NO: 67 - DNA, 28 bp, Artificial Sequence
  Description of Artificial Sequence: Synthetic probe
  5' amino modifier C6
cccaagtagctttgctctactcgtaaaa

SEQ ID NO: 68 - DNA, 28 bp, Artificial Sequence
  Description of Artificial Sequence: Synthetic probe
  5' amino modifier C6
cccaacttcgaactaaggagtagagcaa

SEQ ID NO: 69 - DNA, 28 bp, Artificial Sequence
  Description of Artificial Sequence: Synthetic probe
  5' amino modifier C6
cccaattcagtcctagaggagagactaa

SEQ ID NO: 70 - DNA, 28 bp, Artificial Sequence
  Description of Artificial Sequence: Synthetic probe
  5' amino modifier C6
cccaataggtctgtcttacccaacgtaa

SEQ ID NO: 71 - DNA, 28 bp, Artificial Sequence
  Description of Artificial Sequence: Synthetic probe
  5' amino modifier C6
cccaacgtgaggaaagttctgctaacaa

SEQ ID NO: 72 - DNA, 28 bp, Artificial Sequence
  Description of Artificial Sequence: Synthetic probe
  5' amino modifier C6
cccaagttggcaacttgctctctaagaa

SEQ ID NO: 73 - DNA, 28 bp, Artificial Sequence
  Description of Artificial Sequence: Synthetic probe
  5' amino modifier C6
cccaagacatctctctcagagctagaaa

SEQ ID NO: 74 - DNA, 28 bp, Artificial Sequence
  Description of Artificial Sequence: Synthetic probe
  5' amino modifier C6
cccaatttcgcatgtctcatcaggacaa

SEQ ID NO: 75 - DNA, 28 bp, Artificial Sequence
  Description of Artificial Sequence: Synthetic probe
  5' amino modifier C6
cccaaagccttccttggtactgaaagaa

SEQ ID NO: 76 - DNA, 28 bp, Artificial Sequence
  Description of Artificial Sequence: Synthetic probe
  5' amino modifier C6
cccaaacttgccttgcgtactgtaaaaa

SEQ ID NO: 77 - DNA, 28 bp, Artificial Sequence
  Description of Artificial Sequence: Synthetic probe
  5' amino modifier C6
cccaacactttgtacggtagagacgtaa

SEQ ID NO: 78 - DNA, 28 bp, Artificial Sequence
  Description of Artificial Sequence: Synthetic probe
  5' amino modifier C6
cccaagtttccatcaaccgaagcttgaa

SEQ ID NO: 79 - DNA, 28 bp, Artificial Sequence
  Description of Artificial Sequence: Synthetic probe
  5' amino modifier C6
cccaagcattaccaaactggaacctgaa

SEQ ID NO: 80 - DNA, 28 bp, Artificial Sequence
  Description of Artificial Sequence: Synthetic probe
  5' amino modifier C6
cccaaccgtacaacttgttcgtttgaaa

SEQ ID NO: 81 - DNA, 28 bp, Artificial Sequence
  Description of Artificial Sequence: Synthetic probe
  5' amino modifier C6
cccaacagctagtagcacaccatttgaa

SEQ ID NO: 82 - DNA, 28 bp, Artificial Sequence
  Description of Artificial Sequence: Synthetic probe
  5' amino modifier C6
cccaacctcacgaaagcatcattgtgaa

SEQ ID NO: 83 - DNA, 28 bp, Artificial Sequence
  Description of Artificial Sequence: Synthetic probe
  5' amino modifier C6
cccaaacaaagtgaggtcatctcgacaa

SEQ ID NO: 84 - DNA, 28 bp, Artificial Sequence
  Description of Artificial Sequence: Synthetic probe
  5' amino modifier C6
cccaagaaaccttcttgtaggactcgaa

SEQ ID NO: 85 - DNA, 28 bp, Artificial Sequence
  Description of Artificial Sequence: Synthetic probe
  5' amino modifier C6
cccaaaagcctaagctctgtcagtttaa

SEQ ID NO: 86 - DNA, 28 bp, Artificial Sequence
  Description of Artificial Sequence: Synthetic probe
  5' amino modifier C6
cccaaacgttcccttcatgtcgaaagaa

SEQ ID NO: 87 - DNA, 28 bp, Artificial Sequence
  Description of Artificial Sequence: Synthetic probe
  5' amino modifier C6
cccaagtagcactgacaccaagcattaa

SEQ ID NO: 88 - DNA, 28 bp, Artificial Sequence
  Description of Artificial Sequence: Synthetic probe
  5' amino modifier C6
cccaagtttgactccaagcctacgtcaa

SEQ ID NO: 89 - DNA, 28 bp, Artificial Sequence
  Description of Artificial Sequence: Synthetic probe
  5' amino modifier C6
cccaaaccgttggtgaagccttaaagaa

SEQ ID NO: 90 - DNA, 28 bp, Artificial Sequence
  Description of Artificial Sequence: Synthetic probe
  5' amino modifier C6
cccaagcctacaccttcagtgaacagaa

SEQ ID NO: 91 - DNA, 28 bp, Artificial Sequence
  Description of Artificial Sequence: Synthetic probe
  5' amino modifier C6
cccaacagctcaagcagttagtaaacaa

SEQ ID NO: 92 - DNA, 28 bp, Artificial Sequence
  Description of Artificial Sequence: Synthetic probe
  5' amino modifier C6
cccaatacgcaagcatgtaggtttacaa

SEQ ID NO: 93 - DNA, 28 bp, Artificial Sequence
  Description of Artificial Sequence: Synthetic probe
  5' amino modifier C6
cccaacacgagtcgttagttgtttcaaa

SEQ ID NO: 94 - DNA, 28 bp, Artificial Sequence
  Description of Artificial Sequence: Synthetic probe
  5' amino modifier C6
cccaattcggaagacctactaacctgaa

SEQ ID NO: 95 - DNA, 28 bp, Artificial Sequence
  Description of Artificial Sequence: Synthetic probe
  5' amino modifier C6
cccaaaggtctctacgaaaggaacataa

SEQ ID NO: 96 - DNA, 28 bp, Artificial Sequence
  Description of Artificial Sequence: Synthetic probe
  5' amino modifier C6
cccaagtgctagacgtctgtgtcaaaaa

SEQ ID NO: 97 - DNA, 28 bp, Artificial Sequence
  Description of Artificial Sequence: Synthetic probe
  5' amino modifier C6
cccaaaccagtggacttctctcctagaa

SEQ ID NO: 98 - DNA, 28 bp, Artificial Sequence
  Description of Artificial Sequence: Synthetic probe
  5' amino modifier C6
cccaacatgtaggagacgtagttcccaa

SEQ ID NO: 99 - DNA, 28 bp, Artificial Sequence
  Description of Artificial Sequence: Synthetic probe
  5' amino modifier C6
cccaagaactctctggttaggcttgaaa

SEQ ID NO: 100 - DNA, 28 bp, Artificial Sequence
  Description of Artificial Sequence: Synthetic probe
  5' amino modifier C6
cccaaggacatccacatcgtctgacaaa

SEQ ID NO: 101 - DNA, 28 bp, Artificial Sequence
  Description of Artificial Sequence: Synthetic probe
  5' amino modifier C6
cccaaacttgttgggttcagctaacaaa

SEQ ID NO: 102 - DNA, 28 bp, Artificial Sequence
  Description of Artificial Sequence: Synthetic probe
  5' amino modifier C6
cccaacacgtgtcctgtcatgtcaaaaa

SEQ ID NO: 103 - DNA, 28 bp, Artificial Sequence
  Description of Artificial Sequence: Synthetic probe
  5' amino modifier C6
cccaatcggaaaccaacgttagctttaa

SEQ ID NO: 104 - DNA, 28 bp, Artificial Sequence
  Description of Artificial Sequence: Synthetic probe
  5' amino modifier C6
cccaaggacttaggtacctgttcggaaa

SEQ ID NO: 105 - DNA, 28 bp, Artificial Sequence
  Description of Artificial Sequence: Synthetic probe
  5' amino modifier C6
cccaagacttaacaacctgtgacgagaa

SEQ ID NO: 106 - DNA, 28 bp, Artificial Sequence
  Description of Artificial Sequence: Synthetic probe
  5' amino modifier C6
cccaagttaacatgcagacgaacggtaa

SEQ ID NO: 107 - DNA, 28 bp, Artificial Sequence
  Description of Artificial Sequence: Synthetic probe
  5' amino modifier C6
cccaagcgtacaactcttgtcagtttaa

SEQ ID NO: 108 - DNA, 28 bp, Artificial Sequence
  Description of Artificial Sequence: Synthetic probe
  5' amino modifier C6
cccaagtaacaccttctgagcagtggaa

SEQ ID NO: 109 - DNA, 28 bp, Artificial Sequence
  Description of Artificial Sequence: Synthetic probe
  5' amino modifier C6
cccaagacctacctctcaggaacagtaa

SEQ ID NO: 110 - DNA, 28 bp, Artificial Sequence
  Description of Artificial Sequence: Synthetic probe
  5' amino modifier C6
cccaaacctgaccttaggaagagcataa

SEQ ID NO: 111 - DNA, 28 bp, Artificial Sequence
  Description of Artificial Sequence: Synthetic probe
  5' amino modifier C6
cccaacaaagtttgtctcagttagcgaa

SEQ ID NO: 112 - DNA, 28 bp, Artificial Sequence
  Description of Artificial Sequence: Synthetic probe
  5' amino modifier C6
cccaacggtagcattgttcctgtagaaa

SEQ ID NO: 113 - DNA, 28 bp, Artificial Sequence
  Description of Artificial Sequence: Synthetic probe
  5' amino modifier C6
cccaactaggtttgttctagacagctaa

SEQ ID NO: 114 - DNA, 28 bp, Artificial Sequence
  Description of Artificial Sequence: Synthetic probe
  5' amino modifier C6
cccaagtctctacgttccatcgaaagaa

SEQ ID NO: 115 - DNA, 28 bp, Artificial Sequence
  Description of Artificial Sequence: Synthetic probe
  5' amino modifier C6
cccaaaccttcgttcttgagtacagcaa

SEQ ID NO: 116 - DNA, 28 bp, Artificial Sequence
  Description of Artificial Sequence: Synthetic probe
  5' amino modifier C6
cccaagaacactcctcatgtgactgcaa

SEQ ID NO: 117 - DNA, 28 bp, Artificial Sequence
  Description of Artificial Sequence: Synthetic probe
  5' amino modifier C6
cccaaacgcttggtaacaaagacagtaa

SEQ ID NO: 118 - DNA, 28 bp, Artificial Sequence
  Description of Artificial Sequence: Synthetic probe
  5' amino modifier C6
cccaaccctagagtagtactacggttaa

SEQ ID NO: 119 - DNA, 28 bp, Artificial Sequence
  Description of Artificial Sequence: Synthetic probe
  5' amino modifier C6
cccaacctgaggtagtgactgaaacaaa

SEQ ID NO: 120 - DNA, 28 bp, Artificial Sequence
  Description of Artificial Sequence: Synthetic probe
  5' amino modifier C6
cccaagctacgaacttggttgtttcaaa

SEQ ID NO: 121 - DNA, 28 bp, Artificial Sequence
  Description of Artificial Sequence: Synthetic probe
  5' amino modifier C6
cccaagcaagtcctaggttgtgttcaaa

SEQ ID NO: 122 - DNA, 28 bp, Artificial Sequence
  Description of Artificial Sequence: Synthetic probe
  5' amino modifier C6
cccaactccatgtcaaggaagggtacaa

SEQ ID NO: 123 - DNA, 28 bp, Artificial Sequence
  Description of Artificial Sequence: Synthetic probe
  5' amino modifier C6
cccaatccgaacacgaagtacaagttaa

SEQ ID NO: 124 - DNA, 28 bp, Artificial Sequence
  Description of Artificial Sequence: Synthetic probe
  5' amino modifier C6
cccaacacgttgacattgttggcttaaa

SEQ ID NO: 125 - DNA, 28 bp, Artificial Sequence
  Description of Artificial Sequence: Synthetic probe
  5' amino modifier C6
cccaacctctaggaacgtagtacaccaa

SEQ ID NO: 126 - DNA, 28 bp, Artificial Sequence
  Description of Artificial Sequence: Synthetic probe
  5' amino modifier C6
cccaataggacaccacagttcatcgaaa

SEQ ID NO: 127 - DNA, 28 bp, Artificial Sequence
  Description of Artificial Sequence: Synthetic probe
  5' amino modifier C6
cccaaatgtcgttcggttagctcaaaaa

SEQ ID NO: 128 - DNA, 28 bp, Artificial Sequence
  Description of Artificial Sequence: Synthetic probe
  5' amino modifier C6
cccaaatcggttgtgtctagctcaaaaa

SEQ ID NO: 129 - DNA, 28 bp, Artificial Sequence
  Description of Artificial Sequence: Synthetic probe
  5' amino modifier C6
cccaataagaacgaaacgtaccttgcaa

SEQ ID NO: 130 - DNA, 28 bp, Artificial Sequence
  Description of Artificial Sequence: Synthetic probe
  5' amino modifier C6
cccaatcgcaagaaccgttagtcaaaaa

SEQ ID NO: 131 - DNA, 28 bp, Artificial Sequence
  Description of Artificial Sequence: Synthetic probe
  5' amino modifier C6
cccaagtcacacgtctccacaggtttaa

SEQ ID NO: 132 - DNA, 28 bp, Artificial Sequence
  Description of Artificial Sequence: Synthetic probe
  5' amino modifier C6
cccaagagcttacatcgttctagggtaa

SEQ ID NO: 133 - DNA, 28 bp, Artificial Sequence
  Description of Artificial Sequence: Synthetic probe
  5' amino modifier C6
cccaagaccttctccttgacagaggtaa

SEQ ID NO: 134 - DNA, 28 bp, Artificial Sequence
  Description of Artificial Sequence: Synthetic probe
  5' amino modifier C6
cccaaaaggcttagctctctttactgaa

SEQ ID NO: 135 - DNA, 28 bp, Artificial Sequence
  Description of Artificial Sequence: Synthetic probe
  5' amino modifier C6
cccaagtcgtaacagaggtgtccacaaa

SEQ ID NO: 136 - DNA, 28 bp, Artificial Sequence
  Description of Artificial Sequence: Synthetic probe
  5' amino modifier C6
cccaaactactgcaagtggtaggttcaa

SEQ ID NO: 137 - DNA, 28 bp, Artificial Sequence
  Description of Artificial Sequence: Synthetic probe
  5' amino modifier C6
cccaatttcggaaccagtaccatgggaa

SEQ ID NO: 138 - DNA, 28 bp, Artificial Sequence
  Description of Artificial Sequence: Synthetic probe
  5' amino modifier C6
cccaatcgagaagcaacttccttgtaaa

SEQ ID NO: 139 - DNA, 28 bp, Artificial Sequence
  Description of Artificial Sequence: Synthetic probe
  5' amino modifier C6
cccaatggagacttccgtactgttgaaa

SEQ ID NO: 140 - DNA, 28 bp, Artificial Sequence
  Description of Artificial Sequence: Synthetic probe
  5' amino modifier C6
cccaaacatgcgtttcgtagtcttcaaa

SEQ ID NO: 141 - DNA, 28 bp, Artificial Sequence
  Description of Artificial Sequence: Synthetic probe
  5' amino modifier C6
cccaagaacctcagctctttcgaaagaa

SEQ ID NO: 142 - DNA, 28 bp, Artificial Sequence
  Description of Artificial Sequence: Synthetic probe
  5' amino modifier C6
cccaagtccttaagctgttcgagagtaa

SEQ ID NO: 143 - DNA, 28 bp, Artificial Sequence
  Description of Artificial Sequence: Synthetic probe
  5' amino modifier C6
cccaatctcgaaactcttgtgtgaccaa

SEQ ID NO: 144 - DNA, 28 bp, Artificial Sequence
  Description of Artificial Sequence: Synthetic probe
  5' amino modifier C6
cccaaccattagaggaactaagagctaa

SEQ ID NO: 145 - DNA, 28 bp, Artificial Sequence
  Description of Artificial Sequence: Synthetic probe
  5' amino modifier C6
cccaaccctagagtgagtcaggaactaa

SEQ ID NO: 146 - DNA, 28 bp, Artificial Sequence
  Description of Artificial Sequence: Synthetic probe
  5' amino modifier C6
cccaatgaaccataagagcaacggttaa

SEQ ID NO: 147 - DNA, 28 bp, Artificial Sequence
  Description of Artificial Sequence: Synthetic probe
  5' amino modifier C6
cccaagaaccttcccttagtcgttgaaa

SEQ ID NO: 148 - DNA, 28 bp, Artificial Sequence
  Description of Artificial Sequence: Synthetic probe
  5' amino modifier C6
cccaagtggtcagtaaccctttccgaaa

SEQ ID NO: 149 - DNA, 28 bp, Artificial Sequence
  Description of Artificial Sequence: Synthetic probe
  5' amino modifier C6
cccaaagcatgtacgtctcctactagaa

SEQ ID NO: 150 - DNA, 28 bp, Artificial Sequence
  Description of Artificial Sequence: Synthetic probe
  5' amino modifier C6
cccaaggacttcacctacgttcgaacaa

SEQ ID NO: 151 - DNA, 28 bp, Artificial Sequence
  Description of Artificial Sequence: Synthetic probe
  5' amino modifier C6
cccaacgaactttaccttgtccatggaa

SEQ ID NO: 152 - DNA, 28 bp, Artificial Sequence
  Description of Artificial Sequence: Synthetic probe
  5' amino modifier C6
cccaacaggttcttacgcaacacatgaa

SEQ ID NO: 153 - DNA, 28 bp, Artificial Sequence
  Description of Artificial Sequence: Synthetic probe
  5' amino modifier C6
cccaacttgttagggtagctgactcaaa

SEQ ID NO: 154 - DNA, 28 bp, Artificial Sequence
  Description of Artificial Sequence: Synthetic probe
  5' amino modifier C6
cccaactggagaagagactacctgttaa

SEQ ID NO: 155 - DNA, 28 bp, Artificial Sequence
  Description of Artificial Sequence: Synthetic probe
  5' amino modifier C6
cccaactaaggtttggtcagtcctgaaa

SEQ ID NO: 156 - DNA, 28 bp, Artificial Sequence
  Description of Artificial Sequence: Synthetic probe
  5' amino modifier C6
cccaagcacactagcctttctgaaagaa

SEQ ID NO: 157 - DNA, 28 bp, Artificial Sequence
  Description of Artificial Sequence: Synthetic probe
  5' amino modifier C6
cccaagtcctgacgagagtttggtacaa

SEQ ID NO: 158 - DNA, 28 bp, Artificial Sequence
  Description of Artificial Sequence: Synthetic probe
  5' amino modifier C6
cccaatcccaagagtctctggttgacaa

SEQ ID NO: 159 - DNA, 28 bp, Artificial Sequence
  Description of Artificial Sequence: Synthetic probe
  5' amino modifier C6
cccaaggcattcagcattcattcttgaa

SEQ ID NO: 160 - DNA, 28 bp, Artificial Sequence
  Description of Artificial Sequence: Synthetic probe
  5' amino modifier C6
cccaagtttgactaccaagcaactgcaa

SEQ ID NO: 161 - DNA, 28 bp, Artificial Sequence
  Description of Artificial Sequence: Synthetic probe
  5' amino modifier C6
cccaaccttaagctaagtgtgagacgaa

SEQ ID NO: 162 - DNA, 28 bp, Artificial Sequence
  Description of Artificial Sequence: Synthetic probe
  5' amino modifier C6
cccaacttacagctagtttgaagtgcaa

SEQ ID NO: 163 - DNA, 28 bp, Artificial Sequence
  Description of Artificial Sequence: Synthetic probe
  5' amino modifier C6
cccaactagtctcttagagtttggcaaa

SEQ ID NO: 164 - DNA, 28 bp, Artificial Sequence
  Description of Artificial Sequence: Synthetic probe
  5' amino modifier C6
cccaataaagctctaggagaacacgtaa

SEQ ID NO: 165 - DNA, 28 bp, Artificial Sequence
  Description of Artificial Sequence: Synthetic probe
  5' amino modifier C6
cccaaagcgtagtagtgactaacgacaa

SEQ ID NO: 166 - DNA, 28 bp, Artificial Sequence
  Description of Artificial Sequence: Synthetic probe
  5' amino modifier C6
cccaagacgtaaacgcttccttctagaa

SEQ ID NO: 167 - DNA, 28 bp, Artificial Sequence
  Description of Artificial Sequence: Synthetic probe
  5' amino modifier C6
cccaaagctgtagtaccctttcctagaa

SEQ ID NO: 168 - DNA, 28 bp, Artificial Sequence
  Description of Artificial Sequence: Synthetic probe
  5' amino modifier C6
cccaactcgtacagcatacctagaagaa

SEQ ID NO: 169 - DNA, 28 bp, Artificial Sequence
  Description of Artificial Sequence: Synthetic probe
  5' amino modifier C6
cccaatcgctacatagcaactgaaagaa

SEQ ID NO: 170 - DNA, 28 bp, Artificial Sequence
  Description of Artificial Sequence: Synthetic probe
  5' amino modifier C6
cccaacttggcaacgtgtgtagtacaaa

SEQ ID NO: 171 - DNA, 28 bp, Artificial Sequence
  Description of Artificial Sequence: Synthetic probe
  5' amino modifier C6
cccaaacctgttacgcttgtgctaaaaa

SEQ ID NO: 172 - DNA, 28 bp, Artificial Sequence
  Description of Artificial Sequence: Synthetic probe
  5' amino modifier C6
cccaaagcttggttgtaactttaccgaa

SEQ ID NO: 173 - DNA, 28 bp, Artificial Sequence
  Description of Artificial Sequence: Synthetic probe
  5' amino modifier C6
cccaagagaccttagcaacaaccttgaa

SEQ ID NO: 174 - DNA, 28 bp, Artificial Sequence
  Description of Artificial Sequence: Synthetic probe
  5' amino modifier C6
cccaataccgaagagtgctaggtttcaa

SEQ ID NO: 175 - DNA, 28 bp, Artificial Sequence
  Description of Artificial Sequence: Synthetic probe
  5' amino modifier C6
cccaagacatagtaccgttgctacccaa

SEQ ID NO: 176 - DNA, 28 bp, Artificial Sequence
  Description of Artificial Sequence: Synthetic probe
  5' amino modifier C6
cccaaggtctagtaacgaagcaacctaa

SEQ ID NO: 177 - DNA, 28 bp, Artificial Sequence
  Description of Artificial Sequence: Synthetic probe
  5' amino modifier C6
cccaataagcaacaaaggtcattgccaa

SEQ ID NO: 178 - DNA, 28 bp, Artificial Sequence
  Description of Artificial Sequence: Synthetic probe
  5' amino modifier C6
cccaactgagtgagaagtcagaacctaa

SEQ ID NO: 179 - DNA, 28 bp, Artificial Sequence
  Description of Artificial Sequence: Synthetic probe
  5' amino modifier C6
cccaacttcgagtgaaacaagaacctaa

SEQ ID NO: 180 - DNA, 28 bp, Artificial Sequence
  Description of Artificial Sequence: Synthetic probe
  5' amino modifier C6
cccaaagcgttcatggttctgtcataaa

SEQ ID NO: 181 - DNA, 28 bp, Artificial Sequence
  Description of Artificial Sequence: Synthetic probe
  5' amino modifier C6
cccaagaggtctaggctttcgtctaaaa

SEQ ID NO: 182 - DNA, 28 bp, Artificial Sequence
  Description of Artificial Sequence: Synthetic probe
  5' amino modifier C6
cccaaagccattagtcgtgtcgttacaa

SEQ ID NO: 183 - DNA, 28 bp, Artificial Sequence
  Description of Artificial Sequence: Synthetic probe
  5' amino modifier C6
cccaaggtcttacgtaggttgaagccaa

SEQ ID NO: 184 - DNA, 28 bp, Artificial Sequence
  Description of Artificial Sequence: Synthetic probe
  5' amino modifier C6
cccaagagcttagcgaacttagaaccaa

SEQ ID NO: 185 - DNA, 28 bp, Artificial Sequence
  Description of Artificial Sequence: Synthetic probe
  5' amino modifier C6
cccaatggaaccctagggttgagttcaa

SEQ ID NO: 186 - DNA, 28 bp, Artificial Sequence
  Description of Artificial Sequence: Synthetic probe
  5' amino modifier C6
cccaagaacacttgagcagacgtttcaa

SEQ ID NO: 187 - DNA, 28 bp, Artificial Sequence
  Description of Artificial Sequence: Synthetic probe
  5' amino modifier C6
cccaatcgaaggaaagcatgactctaaa

SEQ ID NO: 188 - DNA, 28 bp, Artificial Sequence
  Description of Artificial Sequence: Synthetic probe
  5' amino modifier C6
cccaacttagtgagagtgctactcagaa

SEQ ID NO: 189 - DNA, 28 bp, Artificial Sequence
  Description of Artificial Sequence: Synthetic probe
  5' amino modifier C6
cccaaacttgttgaagtgcttcacagaa

SEQ ID NO: 190 - DNA, 28 bp, Artificial Sequence
  Description of Artificial Sequence: Synthetic probe
  5' amino modifier C6
cccaagtgctaacactgttctccatgaa

SEQ ID NO: 191 - DNA, 28 bp, Artificial Sequence
  Description of Artificial Sequence: Synthetic probe
  5' amino modifier C6
cccaacccttagacctgaacatcgtgaa

SEQ ID NO: 192 - DNA, 28 bp, Artificial Sequence
  Description of Artificial Sequence: Synthetic probe
  5' amino modifier C6
cccaacttaaagggtagacctagtcgaa

SEQ ID NO: 193 - DNA, 28 bp, Artificial Sequence
  Description of Artificial Sequence: Synthetic probe
  5' amino modifier C6
cccaaggcatagacctgtcgttcttaaa

SEQ ID NO: 194 - DNA, 28 bp, Artificial Sequence
  Description of Artificial Sequence: Synthetic probe
  5' amino modifier C6
cccaaagcgtttctagggtagtaaccaa

SEQ ID NO: 195 - DNA, 28 bp, Artificial Sequence
  Description of Artificial Sequence: Synthetic probe
  5' amino modifier C6
cccaagcaaactttccaagacgttgtaa

SEQ ID NO: 196 - DNA, 28 bp, Artificial Sequence
  Description of Artificial Sequence: Synthetic probe
  5' amino modifier C6
cccaatctggtaactgctttcgaaccaa

SEQ ID NO: 197 - DNA, 28 bp, Artificial Sequence
  Description of Artificial Sequence: Synthetic probe
  5' amino modifier C6
cccaatcaggagagcaagtactagtcaa

SEQ ID NO: 198 - DNA, 28 bp, Artificial Sequence
  Description of Artificial Sequence: Synthetic probe
  5' amino modifier C6
cccaaacattgtgtcgttaacgcttcaa

SEQ ID NO: 199 - DNA, 28 bp, Artificial Sequence
  Description of Artificial Sequence: Synthetic probe
  5' amino modifier C6
cccaagaggtacttaggcataaccgtaa

SEQ ID NO: 200 - DNA, 28 bp, Artificial Sequence
  Description of Artificial Sequence: Synthetic probe
  5' amino modifier C6
cccaaaaacggtttggcaaactgaccaa

SEQ ID NO: 201 - DNA, 28 bp, Artificial Sequence
  Description of Artificial Sequence: Synthetic probe
  5' amino modifier C6
cccaacataaggcaagggtactgtccaa

SEQ ID NO: 202 - DNA, 28 bp, Artificial Sequence
  Description of Artificial Sequence: Synthetic probe
  5' amino modifier C6
cccaaatgacgacaggagtagtgtccaa

SEQ ID NO: 203 - DNA, 28 bp, Artificial Sequence
  Description of Artificial Sequence: Synthetic probe
  5' amino modifier C6
cccaagacctttgcgtttacaggactaa

SEQ ID NO: 204 - DNA, 28 bp, Artificial Sequence
  Description of Artificial Sequence: Synthetic probe
  5' amino modifier C6
cccaagtctagagtcaacacagcactaa

SEQ ID NO: 205 - DNA, 28 bp, Artificial Sequence
  Description of Artificial Sequence: Synthetic probe
  5' amino modifier C6
cccaagagagcttaaccagactgtccaa

SEQ ID NO: 206 - DNA, 28 bp, Artificial Sequence
  Description of Artificial Sequence: Synthetic probe
  5' amino modifier C6
cccaagaccatactgcacattaggctaa

SEQ ID NO: 207 - DNA, 28 bp, Artificial Sequence
  Description of Artificial Sequence: Synthetic probe
  5' amino modifier C6
cccaagccaactacgtcatagtggtcaa

SEQ ID NO: 208 - DNA, 28 bp, Artificial Sequence
  Description of Artificial Sequence: Synthetic probe
  5' amino modifier C6
cccaatgtcgaacgtaccaagaccataa

SEQ ID NO: 209 - DNA, 28 bp, Artificial Sequence
  Description of Artificial Sequence: Synthetic probe
  5' amino modifier C6
cccaacgtgtaggaagttcgtactcaaa

SEQ ID NO: 210 - DNA, 28 bp, Artificial Sequence
  Description of Artificial Sequence: Synthetic probe
  5' amino modifier C6
cccaaaaaccgtaagccttcatggtgaa

SEQ ID NO: 211 - DNA, 28 bp, Artificial Sequence
  Description of Artificial Sequence: Synthetic probe
  5' amino modifier C6
cccaatcggaaacgcaagttcatgttaa

SEQ ID NO: 212 - DNA, 28 bp, Artificial Sequence
  Description of Artificial Sequence: Synthetic probe
  5' amino modifier C6
cccaatcggtaactagaaagcacagtaa

SEQ ID NO: 213 - DNA, 28 bp, Artificial Sequence
  Description of Artificial Sequence: Synthetic probe
  5' amino modifier C6
cccaagtcgaagtaggctaaagtccaaa

SEQ ID NO: 214 - DNA, 28 bp, Artificial Sequence
  Description of Artificial Sequence: Synthetic probe
  5' amino modifier C6
cccaaacggtagtaccttgtcgtcataa

SEQ ID NO: 215 - DNA, 28 bp, Artificial Sequence
  Description of Artificial Sequence: Synthetic probe
  5' amino modifier C6
cccaacatttggaagttgcatcctgtaa

SEQ ID NO: 216 - DNA, 28 bp, Artificial Sequence
  Description of Artificial Sequence: Synthetic probe
  5' amino modifier C6
cccaacgaagtgttggtcaagtccacaa

SEQ ID NO: 217 - DNA, 28 bp, Artificial Sequence
  Description of Artificial Sequence: Synthetic probe
  5' amino modifier C6
cccaatcaaggaaaggactagttcgcaa

SEQ ID NO: 218 - DNA, 28 bp, Artificial Sequence
  Description of Artificial Sequence: Synthetic probe
  5' amino modifier C6
cccaacgaaacttacaacgtaggactaa

SEQ ID NO: 219 - DNA, 28 bp, Artificial Sequence
  Description of Artificial Sequence: Synthetic probe
  5' amino modifier C6
cccaaggcatgcttagtctgaactttaa

SEQ ID NO: 220 - DNA, 28 bp, Artificial Sequence
  Description of Artificial Sequence: Synthetic probe
  5' amino modifier C6
cccaagaaccgttcccatgtagctttaa

SEQ ID NO: 221 - DNA, 28 bp, Artificial Sequence
  Description of Artificial Sequence: Synthetic probe
  5' amino modifier C6
cccaaggcataaagtgttctctcgaaaa

SEQ ID NO: 222 - DNA, 28 bp, Artificial Sequence
  Description of Artificial Sequence: Synthetic probe
  5' amino modifier C6
cccaaggctacccttaaagaggacataa

SEQ ID NO: 223 - DNA, 28 bp, Artificial Sequence
  Description of Artificial Sequence: Synthetic probe
  5' amino modifier C6
cccaagtcctagacttcggttcgtaaaa

SEQ ID NO: 224 - DNA, 28 bp, Artificial Sequence
  Description of Artificial Sequence: Synthetic probe
  5' amino modifier C6
cccaaggaaccttgtacaacacgactaa

SEQ ID NO: 225 - DNA, 28 bp, Artificial Sequence
  Description of Artificial Sequence: Synthetic probe
  5' amino modifier C6
cccaacacgttgtagagacagagactaa

SEQ ID NO: 226 - DNA, 28 bp, Artificial Sequence
  Description of Artificial Sequence: Synthetic probe
  5' amino modifier C6
cccaatccaagcacaaggtaggtttcaa

SEQ ID NO: 227 - DNA, 28 bp, Artificial Sequence
  Description of Artificial Sequence: Synthetic probe
  5' amino modifier C6
cccaaagccatactagttgttgtcgaaa

SEQ ID NO: 228 - DNA, 28 bp, Artificial Sequence
  Description of Artificial Sequence: Synthetic probe
  5' amino modifier C6
cccaacgagtaccatagtgaaggactaa

SEQ ID NO: 229 - DNA, 28 bp, Artificial Sequence
  Description of Artificial Sequence: Synthetic probe
  5' amino modifier C6
cccaacatttgccaagggtagagactaa

SEQ ID NO: 230 - DNA, 28 bp, Artificial Sequence
  Description of Artificial Sequence: Synthetic probe
  5' amino modifier C6
cccaacgactgtttccgtaaagctttaa

SEQ ID NO: 231 - DNA, 28 bp, Artificial Sequence
  Description of Artificial Sequence: Synthetic probe
  5' amino modifier C6
cccaaggagtacgagacatcaagcttaa

SEQ ID NO: 232 - DNA, 28 bp, Artificial Sequence
  Description of Artificial Sequence: Synthetic probe
  5' amino modifier C6
cccaatggactgtctggagtaacgtcaa

SEQ ID NO: 233 - DNA, 28 bp, Artificial Sequence
  Description of Artificial Sequence: Synthetic probe
  5' amino modifier C6
cccaaaccgttacaggtttagtgtcgaa

SEQ ID NO: 234 - DNA, 28 bp, Artificial Sequence
  Description of Artificial Sequence: Synthetic probe
  5' amino modifier C6
cccaatgacaaagagtacgaactgctaa

SEQ ID NO: 235 - DNA, 28 bp, Artificial Sequence
  Description of Artificial Sequence: Synthetic probe
  5' amino modifier C6
cccaatcacaagtgacaaagtacgctaa

SEQ ID NO: 236 - DNA, 28 bp, Artificial Sequence
  Description of Artificial Sequence: Synthetic probe
  5' amino modifier C6
cccaactgtaaagagttgctagctctaa

SEQ ID NO: 237 - DNA, 28 bp, Artificial Sequence
  Description of Artificial Sequence: Synthetic probe
  5' amino modifier C6
cccaatgggaacactgtgaagtcgacaa

SEQ ID NO: 238 - DNA, 28 bp, Artificial Sequence
  Description of Artificial Sequence: Synthetic probe
  5' amino modifier C6
cccaaattgcgtttggtcaactggacaa

SEQ ID NO: 239 - DNA, 28 bp, Artificial Sequence
  Description of Artificial Sequence: Synthetic probe
  5' amino modifier C6
cccaacgaaggttcaggttagtccacaa

SEQ ID NO: 240 - DNA, 28 bp, Artificial Sequence
  Description of Artificial Sequence: Synthetic probe
  5' amino modifier C6
cccaaatgctgtgttaacctttagccaa

SEQ ID NO: 241 - DNA, 28 bp, Artificial Sequence
  Description of Artificial Sequence: Synthetic probe
  5' amino modifier C6
cccaaccacttgtagtactaggttcgaa

SEQ ID NO: 242 - DNA, 28 bp, Artificial Sequence
  Description of Artificial Sequence: Synthetic probe
  5' amino modifier C6
cccaacccatagaggtttcacgttgtaa

SEQ ID NO: 243 - DNA, 28 bp, Artificial Sequence
  Description of Artificial Sequence: Synthetic probe
  5' amino modifier C6
cccaactaggaaagagttcaacgcataa

SEQ ID NO: 244 - DNA, 28 bp, Artificial Sequence
  Description of Artificial Sequence: Synthetic probe
  5' amino modifier C6
cccaatccgaagaaaggtctacaggtaa

SEQ ID NO: 245 - DNA, 28 bp, Artificial Sequence
  Description of Artificial Sequence: Synthetic probe
  5' amino modifier C6
cccaatggaaacccttaagaactgctaa

SEQ ID NO: 246 - DNA, 28 bp, Artificial Sequence
  Description of Artificial Sequence: Synthetic probe
  5' amino modifier C6
cccaagcaacataaccttgactcaggaa

SEQ ID NO: 247 - DNA, 28 bp, Artificial Sequence
  Description of Artificial Sequence: Synthetic probe
  5' amino modifier C6
cccaatagaaccacagactttagcagaa

SEQ ID NO: 248 - DNA, 28 bp, Artificial Sequence
  Description of Artificial Sequence: Synthetic probe
  5' amino modifier C6
cccaatcacaagaggttcgtacgaaaaa

SEQ ID NO: 249 - DNA, 28 bp, Artificial Sequence
  Description of Artificial Sequence: Synthetic probe
  5' amino modifier C6
cccaaagctttgtctccagtacgaaaaa

SEQ ID NO: 250 - DNA, 28 bp, Artificial Sequence
  Description of Artificial Sequence: Synthetic probe
  5' amino modifier C6
cccaatcggaaggtgttcagtaaaccaa

SEQ ID NO: 251 - DNA, 28 bp, Artificial Sequence
  Description of Artificial Sequence: Synthetic probe
  5' amino modifier C6
cccaaagtgcattccaagaaacgactaa

SEQ ID NO: 252 - DNA, 28 bp, Artificial Sequence
  Description of Artificial Sequence: Synthetic probe
  5' amino modifier C6
cccaagacgtaaccatcgaactcgttaa

SEQ ID NO: 253 - DNA, 28 bp, Artificial Sequence
  Description of Artificial Sequence: Synthetic probe
  5' amino modifier C6
cccaaccgtagaacgttctttgcttaaa

SEQ ID NO: 254 - DNA, 28 bp, Artificial Sequence
  Description of Artificial Sequence: Synthetic probe
  5' amino modifier C6
cccaagagctcaagggttctagaaccaa

SEQ ID NO: 255 - DNA, 28 bp, Artificial Sequence
  Description of Artificial Sequence: Synthetic probe
  5' amino modifier C6
cccaatcggtagttacgagtaaagccaa

SEQ ID NO: 256 - DNA, 28 bp, Artificial Sequence
  Description of Artificial Sequence: Synthetic probe
  5' amino modifier C6
cccaagacaactagctcttggactccaa

SEQ ID NO: 257 - DNA, 28 bp, Artificial Sequence
  Description of Artificial Sequence: Synthetic probe
  5' amino modifier C6
cccaatgacgaaggacacttagacctaa

SEQ ID NO: 258 - DNA, 28 bp, Artificial Sequence
  Description of Artificial Sequence: Synthetic probe
  5' amino modifier C6
cccaaccgtagaacatttgaagccataa

SEQ ID NO: 259 - DNA, 28 bp, Artificial Sequence
  Description of Artificial Sequence: Synthetic probe
  5' amino modifier C6
cccaaccactcgaacatggtaacgtcaa

SEQ ID NO: 260 - DNA, 28 bp, Artificial Sequence
  Description of Artificial Sequence: Synthetic probe
  5' amino modifier C6
cccaatcgaaccgtaaccatttcaggaa

SEQ ID NO: 261 - DNA, 28 bp, Artificial Sequence
  Description of Artificial Sequence: Synthetic probe
  5' amino modifier C6
cccaactagtggttggaacatgcactaa

SEQ ID NO: 262 - DNA, 28 bp, Artificial Sequence
  Description of Artificial Sequence: Synthetic probe
  5' amino modifier C6
cccaagtgcttactgtccatcggaaaaa

SEQ ID NO: 263 - DNA, 28 bp, Artificial Sequence
  Description of Artificial Sequence: Synthetic probe
  5' amino modifier C6
cccaatgagtctgcatctctttcaagaa

SEQ ID NO: 264 - DNA, 28 bp, Artificial Sequence
  Description of Artificial Sequence: Synthetic probe
  5' amino modifier C6
cccaataggacaaagacgtcttaccgaa

SEQ ID NO: 265 - DNA, 28 bp, Artificial Sequence
  Description of Artificial Sequence: Synthetic probe
  5' amino modifier C6
cccaatcataggctaagggaagacctaa

SEQ ID NO: 266 - DNA, 28 bp, Artificial Sequence
  Description of Artificial Sequence: Synthetic probe
  5' amino modifier C6
cccaacagaggtaaagtccagtggtcaa

SEQ ID NO: 267 - DNA, 28 bp, Artificial Sequence
  Description of Artificial Sequence: Synthetic probe
  5' amino modifier C6
cccaagaccactacaacgttgcatgtaa

SEQ ID NO: 268 - DNA, 28 bp, Artificial Sequence
  Description of Artificial Sequence: Synthetic probe
  5' amino modifier C6
cccaatagaccacaagcatcgttaggaa

SEQ ID NO: 269 - DNA, 28 bp, Artificial Sequence
  Description of Artificial Sequence: Synthetic probe
  5' amino modifier C6
cccaagtcactcacctaagttcggtaaa

SEQ ID NO: 270 - DNA, 28 bp, Artificial Sequence
  Description of Artificial Sequence: Synthetic probe
  5' amino modifier C6
cccaagctttcaagtaccacacgagtaa

SEQ ID NO: 271 - DNA, 28 bp, Artificial Sequence
  Description of Artificial Sequence: Synthetic probe
  5' amino modifier C6
cccaagtcacatcctctagggttcgaaa

SEQ ID NO: 272 - DNA, 28 bp, Artificial Sequence
  Description of Artificial Sequence: Synthetic probe
  5' amino modifier C6
cccaaaaacgttcatttggtctgacgaa

SEQ ID NO: 273 - DNA, 28 bp, Artificial Sequence
  Description of Artificial Sequence: Synthetic probe
  5' amino modifier C6
cccaactgtccattcggaacgtgaaaaa

SEQ ID NO: 274 - DNA, 28 bp, Artificial Sequence
  Description of Artificial Sequence: Synthetic probe
  5' amino modifier C6
cccaaagttctttcttcagcaagggtaa

SEQ ID NO: 275 - DNA, 28 bp, Artificial Sequence
  Description of Artificial Sequence: Synthetic probe
  5' amino modifier C6
cccaatagtcctgtcgttagaaccgtaa

SEQ ID NO: 276 - DNA, 28 bp, Artificial Sequence
  Description of Artificial Sequence: Synthetic probe
  5' amino modifier C6
cccaacgtacatcccttagaaacgtgaa

SEQ ID NO: 277 - DNA, 28 bp, Artificial Sequence
  Description of Artificial Sequence: Synthetic probe
  5' amino modifier C6
cccaacggttcagcactttacatttgaa

SEQ ID NO: 278 - DNA, 28 bp, Artificial Sequence
  Description of Artificial Sequence: Synthetic probe
  5' amino modifier C6
cccaatgcgtaaactcgttgtcctacaa

SEQ ID NO: 279 - DNA, 28 bp, Artificial Sequence
  Description of Artificial Sequence: Synthetic probe
  5' amino modifier C6
cccaatcggtaaacctgtttcgcttaaa

SEQ ID NO: 280 - DNA, 28 bp, Artificial Sequence
  Description of Artificial Sequence: Synthetic probe
  5' amino modifier C6
cccaagtgcaagcacaggtgacatttaa

SEQ ID NO: 281 - DNA, 28 bp, Artificial Sequence
  Description of Artificial Sequence: Synthetic probe
  5' amino modifier C6
cccaagggtacagacgagtaactctgaa

SEQ ID NO: 282 - DNA, 28 bp, Artificial Sequence
  Description of Artificial Sequence: Synthetic probe
  5' amino modifier C6
cccaaaccctagtagttctactcgtgaa

SEQ ID NO: 283 - DNA, 28 bp, Artificial Sequence
  Description of Artificial Sequence: Synthetic probe
  5' amino modifier C6
cccaagtaacccttccgtaggacagtaa

SEQ ID NO: 284 - DNA, 28 bp, Artificial Sequence
  Description of Artificial Sequence: Synthetic probe
  5' amino modifier C6
cccaatttagtcactctggtcaaccgaa

SEQ ID NO: 285 - DNA, 28 bp, Artificial Sequence
  Description of Artificial Sequence: Synthetic probe
  5' amino modifier C6
cccaagtacacaacctctggtaacggaa

SEQ ID NO: 286 - DNA, 28 bp, Artificial Sequence
  Description of Artificial Sequence: Synthetic probe
  5' amino modifier C6
cccaacacaagttcaggtaggagtgcaa

SEQ ID NO: 287 - DNA, 28 bp, Artificial Sequence
  Description of Artificial Sequence: Synthetic probe
  5' amino modifier C6
cccaactaaaggtgtttacgcttccaaa

SEQ ID NO: 288 - DNA, 28 bp, Artificial Sequence
  Description of Artificial Sequence: Synthetic probe
  5' amino modifier C6
cccaactgaagttggtctacctgaggaa

SEQ ID NO: 289 - DNA, 28 bp, Artificial Sequence
  Description of Artificial Sequence: Synthetic probe
  5' amino modifier C6
cccaatgtcgtaagttcctcaactgcaa

SEQ ID NO: 290 - DNA, 28 bp, Artificial Sequence
  Description of Artificial Sequence: Synthetic probe
  5' amino modifier C6
cccaaacctgagacctgtgtttcgtaaa

SEQ ID NO: 291 - DNA, 28 bp, Artificial Sequence
  Description of Artificial Sequence: Synthetic probe
  5' amino modifier C6
cccaataggctagctcaaccataaagaa

SEQ ID NO: 292 - DNA, 28 bp, Artificial Sequence
  Description of Artificial Sequence: Synthetic probe
  5' amino modifier C6
cccaagttgacaacgctaccctagacaa

SEQ ID NO: 293 - DNA, 28 bp, Artificial Sequence
  Description of Artificial Sequence: Synthetic probe
  5' amino modifier C6
cccaatcacgaagtgagcttgtcaaaaa

SEQ ID NO: 294 - DNA, 28 bp, Artificial Sequence
  Description of Artificial Sequence: Synthetic probe
  5' amino modifier C6
cccaatgaaaccgtaactcacttggcaa

SEQ ID NO: 295 - DNA, 28 bp, Artificial Sequence
  Description of Artificial Sequence: Synthetic probe
  5' amino modifier C6
cccaacttagcacaaagtgtagaagcaa

SEQ ID NO: 296 - DNA, 28 bp, Artificial Sequence
  Description of Artificial Sequence: Synthetic probe
  5' amino modifier C6
cccaatgcgtagaaccatgtacaaagaa

SEQ ID NO: 297 - DNA, 28 bp, Artificial Sequence
  Description of Artificial Sequence: Synthetic probe
  5' amino modifier C6
cccaagagttgcttcggtactcaaagaa

SEQ ID NO: 298 - DNA, 28 bp, Artificial Sequence
  Description of Artificial Sequence: Synthetic probe
  5' amino modifier C6
cccaagcgtagttcggaaacactaagaa

SEQ ID NO: 299 - DNA, 28 bp, Artificial Sequence
  Description of Artificial Sequence: Synthetic probe
  5' amino modifier C6
cccaaaagagtcttaccgtactaccgaa

SEQ ID NO: 300 - DNA, 28 bp, Artificial Sequence
  Description of Artificial Sequence: Synthetic probe
  5' amino modifier C6
cccaaaaacggtaggtctctgactccaa

SEQ ID NO: 301 - DNA, 28 bp, Artificial Sequence
  Description of Artificial Sequence: Synthetic probe
  5' amino modifier C6
cccaaggtcagttaagccaacccttgaa

SEQ ID NO: 302 - DNA, 28 bp, Artificial Sequence
  Description of Artificial Sequence: Synthetic probe
  5' amino modifier C6
cccaaaccagtctctcagtttacgtgaa

SEQ ID NO: 303 - DNA, 28 bp, Artificial Sequence
  Description of Artificial Sequence: Synthetic probe
  5' amino modifier C6
cccaataagacaaggacttccatgccaa

SEQ ID NO: 304 - DNA, 28 bp, Artificial Sequence
  Description of Artificial Sequence: Synthetic probe
  5' amino modifier C6
cccaagtcgagaacatggaagtccttaa

SEQ ID NO: 305 - DNA, 28 bp, Artificial Sequence
  Description of Artificial Sequence: Synthetic probe
  5' amino modifier C6
cccaatgcagagaaagtacataccgtaa

SEQ ID NO: 306 - DNA, 28 bp, Artificial Sequence
  Description of Artificial Sequence: Synthetic probe
  5' amino modifier C6
cccaagtgcacttaaggacaacaggtaa

SEQ ID NO: 307 - DNA, 28 bp, Artificial Sequence
  Description of Artificial Sequence: Synthetic probe
  5' amino modifier C6
cccaaacctgtcttaaggcatacggtaa

SEQ ID NO: 308 - DNA, 28 bp, Artificial Sequence
  Description of Artificial Sequence: Synthetic probe
  5' amino modifier C6
cccaagtctctaagtaggcatgctgtaa

SEQ ID NO: 309 - DNA, 28 bp, Artificial Sequence
  Description of Artificial Sequence: Synthetic probe
  5' amino modifier C6
cccaacgtctgacattggagagaactaa

SEQ ID NO: 310 - DNA, 28 bp, Artificial Sequence
  Description of Artificial Sequence: Synthetic probe
  5' amino modifier C6
cccaaaaagctcacgtcttggtcttaaa

SEQ ID NO: 311 - DNA, 28 bp, Artificial Sequence
  Description of Artificial Sequence: Synthetic probe
  5' amino modifier C6
cccaagggtaacagacactttagcgtaa

SEQ ID NO: 312 - DNA, 28 bp, Artificial Sequence
  Description of Artificial Sequence: Synthetic probe
  5' amino modifier C6
cccaatgacctacgagtggagagtacaa

SEQ ID NO: 313 - DNA, 28 bp, Artificial Sequence
  Description of Artificial Sequence: Synthetic probe
  5' amino modifier C6
cccaaagcttgcgaaacctaactaagaa

SEQ ID NO: 314 - DNA, 28 bp, Artificial Sequence
  Description of Artificial Sequence: Synthetic probe
  5' amino modifier C6
cccaatgtcgacagaccatacctaagaa

SEQ ID NO: 315 - DNA, 28 bp, Artificial Sequence
  Description of Artificial Sequence: Synthetic probe
  5' amino modifier C6
cccaaggtcaacaagccatacgttccaa

SEQ ID NO: 316 - DNA, 28 bp, Artificial Sequence
  Description of Artificial Sequence: Synthetic probe
  5' amino modifier C6
cccaactggttactacgaacaggagtaa

SEQ ID NO: 317 - DNA, 28 bp, Artificial Sequence
  Description of Artificial Sequence: Synthetic probe
  5' amino modifier C6
cccaatagagacgttactcctaaccgaa

SEQ ID NO: 318 - DNA, 28 bp, Artificial Sequence
  Description of Artificial Sequence: Synthetic probe
  5' amino modifier C6
cccaaagacagttgacaccttagcctaa

SEQ ID NO: 319 - DNA, 28 bp, Artificial Sequence
  Description of Artificial Sequence: Synthetic probe
  5' amino modifier C6
cccaaatcgagagttacaccttaccgaa

SEQ ID NO: 320 - DNA, 28 bp, Artificial Sequence
  Description of Artificial Sequence: Synthetic probe
  5' amino modifier C6
cccaaacaggtttccaagaactagggaa

SEQ ID NO: 321 - DNA, 28 bp, Artificial Sequence
  Description of Artificial Sequence: Synthetic probe
  5' amino modifier C6
cccaagacaggtaggtcttgctagtcaa

SEQ ID NO: 322 - DNA, 28 bp, Artificial Sequence
  Description of Artificial Sequence: Synthetic probe
  5' amino modifier C6
cccaaggagtctcaaccgttaaccagaa

SEQ ID NO: 323 - DNA, 28 bp, Artificial Sequence
  Description of Artificial Sequence: Synthetic probe
  5' amino modifier C6
cccaagaaacgtacgcttctccattgaa

SEQ ID NO: 324 - DNA, 28 bp, Artificial Sequence
  Description of Artificial Sequence: Synthetic probe
  5' amino modifier C6
cccaacttaggaagcactacgtacccaa

SEQ ID NO: 325 - DNA, 28 bp, Artificial Sequence
  Description of Artificial Sequence: Synthetic probe
  5' amino modifier C6
cccaagtaagctacgttcctgtacccaa

SEQ ID NO: 326 - DNA, 28 bp, Artificial Sequence
  Description of Artificial Sequence: Synthetic probe
  5' amino modifier C6
cccaaccaagtaagtggacactggtgaa

SEQ ID NO: 327 - DNA, 28 bp, Artificial Sequence
  Description of Artificial Sequence: Synthetic probe
  5' amino modifier C6
cccaactgtttacagaggtcagcagtaa

SEQ ID NO: 328 - DNA, 28 bp, Artificial Sequence
  Description of Artificial Sequence: Synthetic probe
  5' amino modifier C6
cccaacacgtcttaaagcagagaactaa

SEQ ID NO: 329 - DNA, 28 bp, Artificial Sequence
  Description of Artificial Sequence: Synthetic probe
  5' amino modifier C6
cccaagaggactgtcctacttccatgaa

SEQ ID NO: 330 - DNA, 28 bp, Artificial Sequence
  Description of Artificial Sequence: Synthetic probe
  5' amino modifier C6
cccaagaacatctccactggtcacgtaa

SEQ ID NO: 331 - DNA, 28 bp, Artificial Sequence
  Description of Artificial Sequence: Synthetic probe
  5' amino modifier C6
cccaatgaagcaacaagtggtactccaa

SEQ ID NO: 332 - DNA, 28 bp, Artificial Sequence
  Description of Artificial Sequence: Synthetic probe
  5' amino modifier C6
cccaatccgtaacagtaggagaacgtaa

SEQ ID NO: 333 - DNA, 28 bp, Artificial Sequence
  Description of Artificial Sequence: Synthetic probe
  5' amino modifier C6
cccaaaccgtaggaactaccattctgaa

SEQ ID NO: 334 - DNA, 28 bp, Artificial Sequence
  Description of Artificial Sequence: Synthetic probe
  5' amino modifier C6
cccaaccagttcgttcaaacagactgaa

SEQ ID NO: 335 - DNA, 28 bp, Artificial Sequence
  Description of Artificial Sequence: Synthetic probe
  5' amino modifier C6
cccaagttaaacatccagagctcacgaa

SEQ ID NO: 336 - DNA, 28 bp, Artificial Sequence
  Description of Artificial Sequence: Synthetic probe
  5' amino modifier C6
cccaagtcacacaacctagagcttggaa

SEQ ID NO: 337 - DNA, 28 bp, Artificial Sequence
  Description of Artificial Sequence: Synthetic probe
  5' amino modifier C6
cccaacatgttagggttaccttggcaaa

SEQ ID NO: 338 - DNA, 28 bp, Artificial Sequence
  Description of Artificial Sequence: Synthetic probe
  5' amino modifier C6
cccaagtcaaaggtactccacttccgaa

SEQ ID NO: 339 - DNA, 28 bp, Artificial Sequence
  Description of Artificial Sequence: Synthetic probe
  5' amino modifier C6
cccaagtagaacgtcaaccacttacgaa

SEQ ID NO: 340 - DNA, 28 bp, Artificial Sequence
  Description of Artificial Sequence: Synthetic probe
  5' amino modifier C6
cccaaggagacttgtcctactctacgaa

SEQ ID NO: 341 - DNA, 28 bp, Artificial Sequence
  Description of Artificial Sequence: Synthetic probe
  5' amino modifier C6
cccaatttcgtagtactcacttgcgaaa

SEQ ID NO: 342 - DNA, 28 bp, Artificial Sequence
  Description of Artificial Sequence: Synthetic probe
  5' amino modifier C6
cccaaccttgtactaggaaggaagctaa

SEQ ID NO: 343 - DNA, 28 bp, Artificial Sequence
  Description of Artificial Sequence: Synthetic probe
  5' amino modifier C6
cccaagtcgtagttgtcacactgcacaa

SEQ ID NO: 344 - DNA, 28 bp, Artificial Sequence
  Description of Artificial Sequence: Synthetic probe
  5' amino modifier C6
cccaacgaagttacgtctttcatgccaa

SEQ ID NO: 345 - DNA, 28 bp, Artificial Sequence
  Description of Artificial Sequence: Synthetic probe
  5' amino modifier C6
cccaaaaggcataaggcttgtcatccaa

SEQ ID NO: 346 - DNA, 28 bp, Artificial Sequence
  Description of Artificial Sequence: Synthetic probe
  5' amino modifier C6
cccaagtgtccatacgctttaccgaaaa

SEQ ID NO: 347 - DNA, 28 bp, Artificial Sequence
  Description of Artificial Sequence: Synthetic probe
  5' amino modifier C6
cccaacggttgacaccagttaccaagaa

SEQ ID NO: 348 - DNA, 28 bp, Artificial Sequence
  Description of Artificial Sequence: Synthetic probe
  5' amino modifier C6
cccaagtgtgcaaccagttactcctgaa

SEQ ID NO: 349 - DNA, 28 bp, Artificial Sequence
  Description of Artificial Sequence: Synthetic probe
  5' amino modifier C6
cccaagctgacagactctctttcatgaa

SEQ ID NO: 350 - DNA, 28 bp, Artificial Sequence
  Description of Artificial Sequence: Synthetic probe
  5' amino modifier C6
cccaagaaagctgtacccttctctagaa

SEQ ID NO: 351 - DNA, 28 bp, Artificial Sequence
  Description of Artificial Sequence: Synthetic probe
  5' amino modifier C6
cccaaatgttgctacaagactaaccgaa

SEQ ID NO: 352 - DNA, 28 bp, Artificial Sequence
  Description of Artificial Sequence: Synthetic probe
  5' amino modifier C6
cccaagtctggaagtgctagtacgtcaa

SEQ ID NO: 353 - DNA, 28 bp, Artificial Sequence
  Description of Artificial Sequence: Synthetic probe
  5' amino modifier C6
cccaatcgcaacttcggtacatttgtaa

SEQ ID NO: 354 - DNA, 28 bp, Artificial Sequence
  Description of Artificial Sequence: Synthetic probe
  5' amino modifier C6
cccaacctgtaacattgaagaagcgtaa

SEQ ID NO: 355 - DNA, 28 bp, Artificial Sequence
  Description of Artificial Sequence: Synthetic probe
  5' amino modifier C6
cccaaactgttggaaagctgaacactaa

SEQ ID NO: 356 - DNA, 28 bp, Artificial Sequence
  Description of Artificial Sequence: Synthetic probe
  5' amino modifier C6
cccaagacgtagcttagagagaacctaa

SEQ ID NO: 357 - DNA, 28 bp, Artificial Sequence
  Description of Artificial Sequence: Synthetic probe
  5' amino modifier C6
cccaacattgttgtggaacctcagagaa

SEQ ID NO: 358 - DNA, 28 bp, Artificial Sequence
  Description of Artificial Sequence: Synthetic probe
  5' amino modifier C6
cccaagtggactagcttcctacactgaa

SEQ ID NO: 359 - DNA, 28 bp, Artificial Sequence
  Description of Artificial Sequence: Synthetic probe
  5' amino modifier C6
cccaaaggaactgacattcaacacgtaa

SEQ ID NO: 360 - DNA, 28 bp, Artificial Sequence
  Description of Artificial Sequence: Synthetic probe
  5' amino modifier C6
cccaatgttcgagtccacaactacagaa

SEQ ID NO: 361 - DNA, 28 bp, Artificial Sequence
  Description of Artificial Sequence: Synthetic probe
  5' amino modifier C6
cccaagtaactactcacagagctaggaa

SEQ ID NO: 362 - DNA, 28 bp, Artificial Sequence
  Description of Artificial Sequence: Synthetic probe
  5' amino modifier C6
cccaagaggactcaccagtactttcgaa

SEQ ID NO: 363 - DNA, 28 bp, Artificial Sequence
  Description of Artificial Sequence: Synthetic probe
  5' amino modifier C6
cccaatagcgttgtttctaaccactgaa

SEQ ID NO: 364 - DNA, 28 bp, Artificial Sequence
  Description of Artificial Sequence: Synthetic probe
  5' amino modifier C6
cccaacatttgttagtagcagtcacgaa

SEQ ID NO: 365 - DNA, 28 bp, Artificial Sequence
  Description of Artificial Sequence: Synthetic probe
  5' amino modifier C6
cccaataacagcaagaccttgtagccaa

SEQ ID NO: 366 - DNA, 28 bp, Artificial Sequence
  Description of Artificial Sequence: Synthetic probe
  5' amino modifier C6
cccaagactctccacacgttgaagacaa

SEQ ID NO: 367 - DNA, 28 bp, Artificial Sequence
  Description of Artificial Sequence: Synthetic probe
  5' amino modifier C6
cccaagaactccatcctgttcgacagaa

SEQ ID NO: 368 - DNA, 28 bp, Artificial Sequence
  Description of Artificial Sequence: Synthetic probe
  5' amino modifier C6
cccaaggttctagttccaactaacgcaa

SEQ ID NO: 369 - DNA, 28 bp, Artificial Sequence
  Description of Artificial Sequence: Synthetic probe
  5' amino modifier C6
cccaaagttgcgtttgtcatagacctaa

SEQ ID NO: 370 - DNA, 28 bp, Artificial Sequence
  Description of Artificial Sequence: Synthetic probe
  5' amino modifier C6
cccaacgcttgaggtaaactaaacagaa

SEQ ID NO: 371 - DNA, 28 bp, Artificial Sequence
  Description of Artificial Sequence: Synthetic probe
  5' amino modifier C6
cccaataacgagtagagctctagaccaa

SEQ ID NO: 372 - DNA, 28 bp, Artificial Sequence
  Description of Artificial Sequence: Synthetic probe
  5' amino modifier C6
cccaagtgagtcatagccataagccaaa

SEQ ID NO: 373 - DNA, 28 bp, Artificial Sequence
  Description of Artificial Sequence: Synthetic probe
  5' amino modifier C6
cccaacttacgtgacttccattcaggaa

SEQ ID NO: 374 - DNA, 28 bp, Artificial Sequence
  Description of Artificial Sequence: Synthetic probe
  5' amino modifier C6
cccaaatcagtgactgtctcttcacgaa

SEQ ID NO: 375 - DNA, 28 bp, Artificial Sequence
  Description of Artificial Sequence: Synthetic probe
  5' amino modifier C6
cccaaaggtactgacttccactcctgaa

SEQ ID NO: 376 - DNA, 28 bp, Artificial Sequence
  Description of Artificial Sequence: Synthetic probe
  5' amino modifier C6
cccaatcgacattacaggaagtacggaa

SEQ ID NO: 377 - DNA, 28 bp, Artificial Sequence
  Description of Artificial Sequence: Synthetic probe
  5' amino modifier C6
cccaaccactggttaaacgtaaacggaa

SEQ ID NO: 378 - DNA, 28 bp, Artificial Sequence
  Description of Artificial Sequence: Synthetic probe
  5' amino modifier C6
cccaagttcattccctaagccttggaaa

SEQ ID NO: 379 - DNA, 28 bp, Artificial Sequence
  Description of Artificial Sequence: Synthetic probe
  5' amino modifier C6
cccaagaaactactccatggttagcgaa

SEQ ID NO: 380 - DNA, 28 bp, Artificial Sequence
  Description of Artificial Sequence: Synthetic probe
  5' amino modifier C6
cccaactaagggttaaagcttaccgtaa

SEQ ID NO: 381 - DNA, 28 bp, Artificial Sequence
  Description of Artificial Sequence: Synthetic probe
  5' amino modifier C6
cccaagagacctgtcacactttaacgaa

SEQ ID NO: 382 - DNA, 28 bp, Artificial Sequence
  Description of Artificial Sequence: Synthetic probe
  5' amino modifier C6
cccaatgaacaacaacatgcttacggaa

SEQ ID NO: 383 - DNA, 28 bp, Artificial Sequence
  Description of Artificial Sequence: Synthetic probe
  5' amino modifier C6
cccaatcagaaagcaacattctagggaa

SEQ ID NO: 384 - DNA, 28 bp, Artificial Sequence
  Description of Artificial Sequence: Synthetic probe
  5' amino modifier C6
cccaataggcttgactcattaaaccgaa

SEQ ID NO: 385 - DNA, 28 bp, Artificial Sequence
  Description of Artificial Sequence: Synthetic probe
  5' amino modifier C6
cccaaactggtttgtagtcctaccgaaa

SEQ ID NO: 386 - DNA, 28 bp, Artificial Sequence
  Description of Artificial Sequence: Synthetic probe
  5' amino modifier C6
cccaaacctgacagcttgtttcttagaa

SEQ ID NO: 387 - DNA, 28 bp, Artificial Sequence
  Description of Artificial Sequence: Synthetic probe
  5' amino modifier C6
cccaacttgctacatagagagagtgcaa

SEQ ID NO: 388 - DNA, 28 bp, Artificial Sequence
  Description of Artificial Sequence: Synthetic probe
  5' amino modifier C6
cccaaggtaaaccttccagtctccagaa

SEQ ID NO: 389 - DNA, 28 bp, Artificial Sequence
  Description of Artificial Sequence: Synthetic probe
  5' amino modifier C6
cccaataccaagtacgcaaactgtggaa

SEQ ID NO: 390 - DNA, 28 bp, Artificial Sequence
  Description of Artificial Sequence: Synthetic probe
  5' amino modifier C6
cccaaccgtaaaccttaaggtgtagcaa

SEQ ID NO: 391 - DNA, 28 bp, Artificial Sequence
  Description of Artificial Sequence: Synthetic probe
  5' amino modifier C6
cccaacattgtttcccaaggcatagcaa

SEQ ID NO: 392 - DNA, 28 bp, Artificial Sequence
  Description of Artificial Sequence: Synthetic probe
  5' amino modifier C6
cccaaggtcatcctactagcattgccaa

SEQ ID NO: 393 - DNA, 28 bp, Artificial Sequence
  Description of Artificial Sequence: Synthetic probe
  5' amino modifier C6
cccaagttcaacatcactgctacggtaa

SEQ ID NO: 394 - DNA, 28 bp, Artificial Sequence
  Description of Artificial Sequence: Synthetic probe
  5' amino modifier C6
cccaattcgcatgcatttaaggtgtcaa

SEQ ID NO: 395 - DNA, 28 bp, Artificial Sequence
  Description of Artificial Sequence: Synthetic probe
  5' amino modifier C6
cccaacttagcactagagaaggagtcaa

SEQ ID NO: 396 - DNA, 28 bp, Artificial Sequence
  Description of Artificial Sequence: Synthetic probe
  5' amino modifier C6
cccaagctcaggacagttgagtgttcaa

SEQ ID NO: 397 - DNA, 28 bp, Artificial Sequence
  Description of Artificial Sequence: Synthetic probe
  5' amino modifier C6
cccaagtcctagctaagagtgtgtcaaa

SEQ ID NO: 398 - DNA, 28 bp, Artificial Sequence
  Description of Artificial Sequence: Synthetic probe
  5' amino modifier C6
cccaagctacaagcataagtggttcaaa

SEQ ID NO: 399 - DNA, 28 bp, Artificial Sequence
  Description of Artificial Sequence: Synthetic probe
  5' amino modifier C6
cccaagtcataccaaagctgagacgtaa

SEQ ID NO: 400 - DNA, 28 bp, Artificial Sequence
  Description of Artificial Sequence: Synthetic probe
  5' amino modifier C6
cccaatttagcatagacgagagactcaa

SEQ ID NO: 401 - DNA, 28 bp, Artificial Sequence
  Description of Artificial Sequence: Synthetic probe
  5' amino modifier C6
cccaatttcatgtaacgacagtgagcaa

SEQ ID NO: 402 - DNA, 28 bp, Artificial Sequence
  Description of Artificial Sequence: Synthetic probe
  5' amino modifier C6
cccaatgcacttcgtagagtaagaacaa

SEQ ID NO: 403 - DNA, 28 bp, Artificial Sequence
  Description of Artificial Sequence: Synthetic probe
  5' amino modifier C6
cccaaacgttgtctctgtagtggaacaa

SEQ ID NO: 404 - DNA, 28 bp, Artificial Sequence
  Description of Artificial Sequence: Synthetic probe
  5' amino modifier C6
cccaaccgaagttagcaaacctcatgaa

SEQ ID NO: 405 - DNA, 28 bp, Artificial Sequence
  Description of Artificial Sequence: Synthetic probe
  5' amino modifier C6
cccaacatttagaaggacttcgaacgaa

SEQ ID NO: 406 - DNA, 28 bp, Artificial Sequence
  Description of Artificial Sequence: Synthetic probe
  5' amino modifier C6
cccaagttccaacactcagacaggtcaa

SEQ ID NO: 407 - DNA, 28 bp, Artificial Sequence
  Description of Artificial Sequence: Synthetic probe
  5' amino modifier C6
cccaatgacaacctctcagagtggtcaa

SEQ ID NO: 408 - DNA, 28 bp, Artificial Sequence
  Description of Artificial Sequence: Synthetic probe
  5' amino modifier C6
cccaagcctaggtaggttctggaactaa

SEQ ID NO: 409 - DNA, 28 bp, Artificial Sequence
  Description of Artificial Sequence: Synthetic probe
  5' amino modifier C6
cccaatcgaacacaccatgttactggaa

SEQ ID NO: 410 - DNA, 28 bp, Artificial Sequence
  Description of Artificial Sequence: Synthetic probe
  5' amino modifier C6
cccaatagtctaactgttggcttgcaaa

SEQ ID NO: 411 - DNA, 28 bp, Artificial Sequence
  Description of Artificial Sequence: Synthetic probe
  5' amino modifier C6
cccaaaagctaggtaccttcttaccgaa

SEQ ID NO: 412 - DNA, 28 bp, Artificial Sequence
  Description of Artificial Sequence: Synthetic probe
  5' amino modifier C6
cccaactcagagtacagagagtttgcaa

SEQ ID NO: 413 - DNA, 28 bp, Artificial Sequence
  Description of Artificial Sequence: Synthetic probe
  5' amino modifier C6
cccaagacacgtcataggagtgtagcaa

SEQ ID NO: 414 - DNA, 28 bp, Artificial Sequence
  Description of Artificial Sequence: Synthetic probe
  5' amino modifier C6
cccaattaagcataacgagacagtgcaa

SEQ ID NO: 415 - DNA, 28 bp, Artificial Sequence
  Description of Artificial Sequence: Synthetic probe
  5' amino modifier C6
cccaagtgtccacatgaggtgaaagcaa

SEQ ID NO: 416 - DNA, 28 bp, Artificial Sequence
  Description of Artificial Sequence: Synthetic probe
  5' amino modifier C6
cccaactaaagggttgaacgttccagaa

SEQ ID NO: 417 - DNA, 28 bp, Artificial Sequence
  Description of Artificial Sequence: Synthetic probe
  5' amino modifier C6
cccaaatcgctttctttagtggagacaa

SEQ ID NO: 418 - DNA, 28 bp, Artificial Sequence
  Description of Artificial Sequence: Synthetic probe
  5' amino modifier C6
cccaaaggtcttcactttgtgcacaaaa

SEQ ID NO: 419 - DNA, 28 bp, Artificial Sequence
  Description of Artificial Sequence: Synthetic probe
  5' amino modifier C6
cccaaggcttaaggtgaaccatcgacaa

SEQ ID NO: 420 - DNA, 28 bp, Artificial Sequence
  Description of Artificial Sequence: Synthetic probe
  5' amino modifier C6
cccaactgtagagctaccaacactagaa

SEQ ID NO: 421 - DNA, 28 bp, Artificial Sequence
  Description of Artificial Sequence: Synthetic probe
  5' amino modifier C6
cccaactaagggttgttacgttagccaa

SEQ ID NO: 422 - DNA, 28 bp, Artificial Sequence
  Description of Artificial Sequence: Synthetic probe
  5' amino modifier C6
cccaagtggtactcagctacatcgtcaa

SEQ ID NO: 423 - DNA, 28 bp, Artificial Sequence
  Description of Artificial Sequence: Synthetic probe
  5' amino modifier C6
cccaagtccaaacaccttgagagctcaa

SEQ ID NO: 424 - DNA, 28 bp, Artificial Sequence
  Description of Artificial Sequence: Synthetic probe
  5' amino modifier C6
cccaatcacaagcttagagtggagacaa

SEQ ID NO: 425 - DNA, 28 bp, Artificial Sequence
  Description of Artificial Sequence: Synthetic probe
  5' amino modifier C6
cccaactttgactttggcaactagggaa

SEQ ID NO: 426 - DNA, 28 bp, Artificial Sequence
  Description of Artificial Sequence: Synthetic probe
  5' amino modifier C6
cccaacctcagtctaagggtagtgtcaa

SEQ ID NO: 427 - DNA, 28 bp, Artificial Sequence
  Description of Artificial Sequence: Synthetic probe
  5' amino modifier C6
cccaaacacctgtccagagagtgtacaa

SEQ ID NO: 428 - DNA, 28 bp, Artificial Sequence
  Description of Artificial Sequence: Synthetic probe
  5' amino modifier C6
cccaacatagttgtgaagcatcgctaaa

SEQ ID NO: 429 - DNA, 28 bp, Artificial Sequence
  Description of Artificial Sequence: Synthetic probe
  5' amino modifier C6
cccaaacgtgttgttgtaccctaggaaa

SEQ ID NO: 430 - DNA, 28 bp, Artificial Sequence
  Description of Artificial Sequence: Synthetic probe
  5' amino modifier C6
cccaaactttggtagaaacgtagccaaa

SEQ ID NO: 431 - DNA, 28 bp, Artificial Sequence
  Description of Artificial Sequence: Synthetic probe
  5' amino modifier C6
cccaactcagttgcattaaagtgtgcaa

SEQ ID NO: 432 - DNA, 28 bp, Artificial Sequence
  Description of Artificial Sequence: Synthetic probe
  5' amino modifier C6
cccaaactactgttctggacttcggaaa

SEQ ID NO: 433 - DNA, 28 bp, Artificial Sequence
  Description of Artificial Sequence: Synthetic probe
  5' amino modifier C6
cccaaagagcattaggactgtacgacaa

SEQ ID NO: 434 - DNA, 28 bp, Artificial Sequence
  Description of Artificial Sequence: Synthetic probe
  5' amino modifier C6
cccaacaccatgctgagtggtaagtcaa

SEQ ID NO: 435 - DNA, 28 bp, Artificial Sequence
  Description of Artificial Sequence: Synthetic probe
  5' amino modifier C6
cccaactggaacacgtgtggtagaacaa

SEQ ID NO: 436 - DNA, 28 bp, Artificial Sequence
  Description of Artificial Sequence: Synthetic probe
  5' amino modifier C6
cccaacctcagaactcgttggttaccaa

SEQ ID NO: 437 - DNA, 28 bp, Artificial Sequence
  Description of Artificial Sequence: Synthetic probe
  5' amino modifier C6
cccaatgccataacgcttgtacttgtaa

SEQ ID NO: 438 - DNA, 28 bp, Artificial Sequence
  Description of Artificial Sequence: Synthetic probe
  5' amino modifier C6
cccaaaaccttgtagacaagaagcgtaa

SEQ ID NO: 439 - DNA, 28 bp, Artificial Sequence
  Description of Artificial Sequence: Synthetic probe
  5' amino modifier C6
cccaacacatgttagagacgacaggtaa

SEQ ID NO: 440 - DNA, 28 bp, Artificial Sequence
  Description of Artificial Sequence: Synthetic probe
  5' amino modifier C6
cccaaggtactctaacttgcagtcctaa

SEQ ID NO: 441 - DNA, 28 bp, Artificial Sequence
  Description of Artificial Sequence: Synthetic probe
  5' amino modifier C6
cccaatgccaacctcaagaagtgtacaa

SEQ ID NO: 442 - DNA, 28 bp, Artificial Sequence
  Description of Artificial Sequence: Synthetic probe
  5' amino modifier C6
cccaactaaagttgggaacgcatcacaa

SEQ ID NO: 443 - DNA, 28 bp, Artificial Sequence
  Description of Artificial Sequence: Synthetic probe
  5' amino modifier C6
cccaaggactactccactgtcatcagaa

SEQ ID NO: 444 - DNA, 28 bp, Artificial Sequence
  Description of Artificial Sequence: Synthetic probe
  5' amino modifier C6
cccaagaaccgtagttccttccctagaa

SEQ ID NO: 445 - DNA, 28 bp, Artificial Sequence
  Description of Artificial Sequence: Synthetic probe
  5' amino modifier C6
cccaactttgaggtgagactcgttacaa

SEQ ID NO: 446 - DNA, 28 bp, Artificial Sequence
  Description of Artificial Sequence: Synthetic probe
  5' amino modifier C6
cccaatcagagaagagttcgtcacacaa

SEQ ID NO: 447 - DNA, 28 bp, Artificial Sequence
  Description of Artificial Sequence: Synthetic probe
  5' amino modifier C6
cccaagtttcattcctcagagctgacaa

SEQ ID NO: 448 - DNA, 28 bp, Artificial Sequence
  Description of Artificial Sequence: Synthetic probe
  5' amino modifier C6
cccaagttgtcactcctgagcactacaa

SEQ ID NO: 449 - DNA, 28 bp, Artificial Sequence
  Description of Artificial Sequence: Synthetic probe
  5' amino modifier C6
cccaaaaggttcatcgctttgaccacaa

SEQ ID NO: 450 - DNA, 28 bp, Artificial Sequence
  Description of Artificial Sequence: Synthetic probe
  5' amino modifier C6
cccaatgccaagacttgtggtgttacaa

SEQ ID NO: 451 - DNA, 28 bp, Artificial Sequence
  Description of Artificial Sequence: Synthetic probe
  5' amino modifier C6
cccaaaggcttcggtaacactaacagaa

SEQ ID NO: 452 - DNA, 28 bp, Artificial Sequence
  Description of Artificial Sequence: Synthetic probe
  5' amino modifier C6
cccaacagctagcatggtttggttacaa

SEQ ID NO: 453 - DNA, 28 bp, Artificial Sequence
  Description of Artificial Sequence: Synthetic probe
  5' amino modifier C6
cccaagccattagcctagttgtccacaa

SEQ ID NO: 454 - DNA, 28 bp, Artificial Sequence
  Description of Artificial Sequence: Synthetic probe
  5' amino modifier C6
cccaacggtacaacggttgggtttacaa

SEQ ID NO: 455 - DNA, 28 bp, Artificial Sequence
  Description of Artificial Sequence: Synthetic probe
  5' amino modifier C6
cccaacaccagttggacaggacattcaa

SEQ ID NO: 456 - DNA, 28 bp, Artificial Sequence
  Description of Artificial Sequence: Synthetic probe
  5' amino modifier C6
cccaatctcagactggaagggttgacaa

SEQ ID NO: 457 - DNA, 28 bp, Artificial Sequence
  Description of Artificial Sequence: Synthetic probe
  5' amino modifier C6
cccaagtgtgacgaacctcaaacatgaa

SEQ ID NO: 458 - DNA, 28 bp, Artificial Sequence
  Description of Artificial Sequence: Synthetic probe
  5' amino modifier C6
cccaatgcgtacaggtacataggacaaa

SEQ ID NO: 459 - DNA, 28 bp, Artificial Sequence
  Description of Artificial Sequence: Synthetic probe
  5' amino modifier C6
cccaacagttaaaggacatgagctcaaa

SEQ ID NO: 460 - DNA, 28 bp, Artificial Sequence
  Description of Artificial Sequence: Synthetic probe
  5' amino modifier C6
cccaatccgaaagggttacagttacgaa

SEQ ID NO: 461 - DNA, 28 bp, Artificial Sequence
  Description of Artificial Sequence: Synthetic probe
  5' amino modifier C6
cccaacattgtgaaagtgcagttcccaa

SEQ ID NO: 462 - DNA, 28 bp, Artificial Sequence
  Description of Artificial Sequence: Synthetic probe
  5' amino modifier C6
cccaaaaccatgaggtcacgttacccaa

SEQ ID NO: 463 - DNA, 28 bp, Artificial Sequence
  Description of Artificial Sequence: Synthetic probe
  5' amino modifier C6
cccaatcaaggagaaacgtgtacctcaa

SEQ ID NO: 464 - DNA, 28 bp, Artificial Sequence
  Description of Artificial Sequence: Synthetic probe
  5' amino modifier C6
cccaatcaggagacgactagtaggtcaa

SEQ ID NO: 465 - DNA, 28 bp, Artificial Sequence
  Description of Artificial Sequence: Synthetic probe
  5' amino modifier C6
cccaaggactaggtcacacatctctgaa

SEQ ID NO: 466 - DNA, 28 bp, Artificial Sequence
  Description of Artificial Sequence: Synthetic probe
  5' amino modifier C6
cccaacatagagaggacatcttcgacaa

SEQ ID NO: 467 - DNA, 28 bp, Artificial Sequence
  Description of Artificial Sequence: Synthetic probe
  5' amino modifier C6
cccaacgaactcatccttgtggacacaa

SEQ ID NO: 468 - DNA, 28 bp, Artificial Sequence
  Description of Artificial Sequence: Synthetic probe
  5' amino modifier C6
cccaacagttggtgagttcatgcacaaa

SEQ ID NO: 469 - DNA, 28 bp, Artificial Sequence
  Description of Artificial Sequence: Synthetic probe
  5' amino modifier C6
cccaacataggacaggagtgttgcacaa

SEQ ID NO: 470 - DNA, 28 bp, Artificial Sequence
  Description of Artificial Sequence: Synthetic probe
  5' amino modifier C6
cccaactagtagaagactgcatggacaa

SEQ ID NO: 471 - DNA, 28 bp, Artificial Sequence
  Description of Artificial Sequence: Synthetic probe
  5' amino modifier C6
cccaatagagcaagaacctcagttggaa

SEQ ID NO: 472 - DNA, 28 bp, Artificial Sequence
  Description of Artificial Sequence: Synthetic probe
  5' amino modifier C6
cccaaccatgtggagtttctgaggacaa

SEQ ID NO: 473 - DNA, 28 bp, Artificial Sequence
  Description of Artificial Sequence: Synthetic probe
  5' amino modifier C6
cccaatagacaggacaggtgttcccaaa

SEQ ID NO: 474 - DNA, 28 bp, Artificial Sequence
  Description of Artificial Sequence: Synthetic probe
  5' amino modifier C6
cccaattcggaagccatttctcttagaa

SEQ ID NO: 475 - DNA, 28 bp, Artificial Sequence
  Description of Artificial Sequence: Synthetic probe
  5' amino modifier C6
cccaatcggaacagttcctcattctgaa

SEQ ID NO: 476 - DNA, 28 bp, Artificial Sequence
  Description of Artificial Sequence: Synthetic probe
  5' amino modifier C6
cccaatgaagcagttccatcattctgaa

SEQ ID NO: 477 - DNA, 28 bp, Artificial Sequence
  Description of Artificial Sequence: Synthetic probe
  5' amino modifier C6
cccaacatgtgtcaagggtagctctcaa

SEQ ID NO: 478 - DNA, 28 bp, Artificial Sequence
  Description of Artificial Sequence: Synthetic probe
  5' amino modifier C6
cccaagcctttacaccatgtggaaccaa

SEQ ID NO: 479 - DNA, 28 bp, Artificial Sequence
  Description of Artificial Sequence: Synthetic probe
  5' amino modifier C6
cccaactaactgctgaggtgaggtacaa

SEQ ID NO: 480 - DNA, 28 bp, Artificial Sequence
  Description of Artificial Sequence: Synthetic probe
  5' amino modifier C6
cccaactccaagtcgagtgagttgacaa

SEQ ID NO: 481 - DNA, 28 bp, Artificial Sequence
  Description of Artificial Sequence: Synthetic probe
  5' amino modifier C6
cccaacgagttgagaagctacatgacaa

SEQ ID NO: 482 - DNA, 28 bp, Artificial Sequence
  Description of Artificial Sequence: Synthetic probe
  5' amino modifier C6
cccaatttctgagtgagcaaccctagaa

SEQ ID NO: 483 - DNA, 28 bp, Artificial Sequence
  Description of Artificial Sequence: Synthetic probe
  5' amino modifier C6
cccaagagtacagctacctctccaagaa

SEQ ID NO: 484 - DNA, 28 bp, Artificial Sequence
  Description of Artificial Sequence: Synthetic probe
  5' amino modifier C6
cccaagagcactccacttgtacaaagaa

SEQ ID NO: 485 - DNA, 28 bp, Artificial Sequence
  Description of Artificial Sequence: Synthetic probe
  5' amino modifier C6
cccaagctacatttcttgagtcgactaa

SEQ ID NO: 486 - DNA, 28 bp, Artificial Sequence
  Description of Artificial Sequence: Synthetic probe
  5' amino modifier C6
cccaaaccgtaggactacaacacttgaa

SEQ ID NO: 487 - DNA, 28 bp, Artificial Sequence
  Description of Artificial Sequence: Synthetic probe
  5' amino modifier C6
cccaaattcctgttgtgacgaagtcgaa

SEQ ID NO: 488 - DNA, 28 bp, Artificial Sequence
  Description of Artificial Sequence: Synthetic probe
  5' amino modifier C6
cccaaagttctgtggttcacaagtcgaa

SEQ ID NO: 489 - DNA, 28 bp, Artificial Sequence
  Description of Artificial Sequence: Synthetic probe
  5' amino modifier C6
cccaagtactcgagttccctttaacgaa

SEQ ID NO: 490 - DNA, 28 bp, Artificial Sequence
  Description of Artificial Sequence: Synthetic probe
  5' amino modifier C6
cccaagctgaaggttaacaacaagctaa

SEQ ID NO: 491 - DNA, 28 bp, Artificial Sequence
  Description of Artificial Sequence: Synthetic probe
  5' amino modifier C6
cccaatcgcatggtaaacaaacactgaa

SEQ ID NO: 492 - DNA, 28 bp, Artificial Sequence
  Description of Artificial Sequence: Synthetic probe
  5' amino modifier C6
cccaactggtactaaagccaaactgcaa

SEQ ID NO: 493 - DNA, 28 bp, Artificial Sequence
  Description of Artificial Sequence: Synthetic probe
  5' amino modifier C6
cccaacgttaagaaggtacctagcctaa

SEQ ID NO: 494 - DNA, 28 bp, Artificial Sequence
  Description of Artificial Sequence: Synthetic probe
  5' amino modifier C6
cccaacagtgaaagttgtccttccagaa

SEQ ID NO: 495 - DNA, 28 bp, Artificial Sequence
  Description of Artificial Sequence: Synthetic probe
  5' amino modifier C6
cccaacaggagttgggtaccagtctaaa

SEQ ID NO: 496 - DNA, 28 bp, Artificial Sequence
  Description of Artificial Sequence: Synthetic probe
  5' amino modifier C6
cccaagaaactgtgcaaacactcctgaa

SEQ ID NO: 497 - DNA, 28 bp, Artificial Sequence
  Description of Artificial Sequence: Synthetic probe
  5' amino modifier C6
cccaatcgtagttcgacaaactccagaa

SEQ ID NO: 498 - DNA, 28 bp, Artificial Sequence
  Description of Artificial Sequence: Synthetic probe
  5' amino modifier C6
cccaacaggttagttcacaccatccgaa

SEQ ID NO: 499 - DNA, 28 bp, Artificial Sequence
  Description of Artificial Sequence: Synthetic probe
  5' amino modifier C6
cccaaggtttacgtcactccatccagaa

SEQ ID NO: 500 - DNA, 28 bp, Artificial Sequence
  Description of Artificial Sequence: Synthetic probe
  5' amino modifier C6
cccaagtttaacctcatgctttagcgaa

SEQ ID NO: 501 - DNA, 28 bp, Artificial Sequence
  Description of Artificial Sequence: Synthetic probe
  5' amino modifier C6
cccaatttgtacgttccaacctaggcaa

SEQ ID NO: 502 - DNA, 28 bp, Artificial Sequence
  Description of Artificial Sequence: Synthetic probe
  5' amino modifier C6
cccaaatcgtttgtttccagtaggcaaa

SEQ ID NO: 503 - DNA, 28 bp, Artificial Sequence
  Description of Artificial Sequence: Synthetic probe
  5' amino modifier C6
cccaagcatccttgtcttaactgcagaa

SEQ ID NO: 504 - DNA, 28 bp, Artificial Sequence
  Description of Artificial Sequence: Synthetic probe
  5' amino modifier C6
cccaaactggtaagtcttggctacccaa

SEQ ID NO: 505 - DNA, 28 bp, Artificial Sequence
  Description of Artificial Sequence: Synthetic probe
  5' amino modifier C6
cccaagtccatgtgcaacaccaactgaa

SEQ ID NO: 506 - DNA, 28 bp, Artificial Sequence
  Description of Artificial Sequence: Synthetic probe
  5' amino modifier C6
cccaagtcacaggactcctcaacatgaa

SEQ ID NO: 507 - DNA, 28 bp, Artificial Sequence
  Description of Artificial Sequence: Synthetic probe
  5' amino modifier C6
cccaagtactctcattctgtgcagacaa

SEQ ID NO: 508 - DNA, 28 bp, Artificial Sequence
  Description of Artificial Sequence: Synthetic probe
  5' amino modifier C6
cccaaggttccacactttgtcacgacaa

SEQ ID NO: 509 - DNA, 28 bp, Artificial Sequence
  Description of Artificial Sequence: Synthetic probe
  5' amino modifier C6
cccaaactcgtctgtccataaagtcgaa

SEQ ID NO: 510 - DNA, 28 bp, Artificial Sequence
  Description of Artificial Sequence: Synthetic probe
  5' amino modifier C6
cccaacaaggtgtgttctaccattcgaa

SEQ ID NO: 511 - DNA, 28 bp, Artificial Sequence
  Description of Artificial Sequence: Synthetic probe
  5' amino modifier C6
cccaaactcgtgttgtacttagaacgaa

SEQ ID NO: 512 - DNA, 28 bp, Artificial Sequence
  Description of Artificial Sequence: Synthetic probe
  5' amino modifier C6
cccaaaggcattgtcaacaaaccagtaa

SEQ ID NO: 513 - DNA, 28 bp, Artificial Sequence
  Description of Artificial Sequence: Synthetic probe
  5' amino modifier C6
cccaacagtagttgttaacgactgctaa

SEQ ID NO: 514 - DNA, 28 bp, Artificial Sequence
  Description of Artificial Sequence: Synthetic probe
  5' amino modifier C6
cccaatgctcaggtcaaacaaactagaa

SEQ ID NO: 515 - DNA, 28 bp, Artificial Sequence
  Description of Artificial Sequence: Synthetic probe
  5' amino modifier C6
cccaatgtcgtactttgagtaagcctaa

SEQ ID NO: 516 - DNA, 28 bp, Artificial Sequence
  Description of Artificial Sequence: Synthetic probe
  5' amino modifier C6
cccaaggctagacgaacattaccatgaa

SEQ ID NO: 517 - DNA, 28 bp, Artificial Sequence
  Description of Artificial Sequence: Synthetic probe
  5' amino modifier C6
cccaacgagtgttctagtgttacacgaa

SEQ ID NO: 518 - DNA, 28 bp, Artificial Sequence
  Description of Artificial Sequence: Synthetic probe
  5' amino modifier C6
cccaacaggtttacgtgtgtacagctaa

SEQ ID NO: 519 - DNA, 28 bp, Artificial Sequence
  Description of Artificial Sequence: Synthetic probe
  5' amino modifier C6
cccaaaggttccttccatgtaagctcaa

SEQ ID NO: 520 - DNA, 28 bp, Artificial Sequence
  Description of Artificial Sequence: Synthetic probe
  5' amino modifier C6
cccaaaggctttgctgttacttagacaa

SEQ ID NO: 521 - DNA, 28 bp, Artificial Sequence
  Description of Artificial Sequence: Synthetic probe
  5' amino modifier C6
cccaacaaagtaactgttcgttgcgaaa

SEQ ID NO: 522 - DNA, 28 bp, Artificial Sequence
  Description of Artificial Sequence: Synthetic probe
  5' amino modifier C6
cccaaatgcttggaacttctaactcgaa

SEQ ID NO: 523 - DNA, 28 bp, Artificial Sequence
  Description of Artificial Sequence: Synthetic probe
  5' amino modifier C6
cccaacctgagtactgtgctctgaaaaa

SEQ ID NO: 524 - DNA, 28 bp, Artificial Sequence
  Description of Artificial Sequence: Synthetic probe
  5' amino modifier C6
cccaaggactcaagtcttccttcacgaa

SEQ ID NO: 525 - DNA, 28 bp, Artificial Sequence
  Description of Artificial Sequence: Synthetic probe
  5' amino modifier C6
cccaaagggttccgttcactaacatgaa

SEQ ID NO: 526 - DNA, 28 bp, Artificial Sequence
  Description of Artificial Sequence: Synthetic probe
  5' amino modifier C6
cccaaccagtactgcatttcttggagaa

SEQ ID NO: 527 - DNA, 28 bp, Artificial Sequence
  Description of Artificial Sequence: Synthetic probe
  5' amino modifier C6
cccaacaagcctagttctggttgtacaa

SEQ ID NO: 528 - DNA, 28 bp, Artificial Sequence
  Description of Artificial Sequence: Synthetic probe
  5' amino modifier C6
cccaacagacctacctttgttgtagcaa

SEQ ID NO: 529 - DNA, 28 bp, Artificial Sequence
  Description of Artificial Sequence: Synthetic probe
  5' amino modifier C6
cccaagaacccttctttgactgcaagaa

SEQ ID NO: 530 - DNA, 28 bp, Artificial Sequence
  Description of Artificial Sequence: Synthetic probe
  5' amino modifier C6
cccaaagtcgtttagtcctctgaccaaa

SEQ ID NO: 531 - DNA, 28 bp, Artificial Sequence
  Description of Artificial Sequence: Synthetic probe
  5' amino modifier C6
cccaaagtctcttcgttcaactggagaa

SEQ ID NO: 532 - DNA, 28 bp, Artificial Sequence
  Description of Artificial Sequence: Synthetic probe
  5' amino modifier C6
cccaacgcattcttaacagagacagtaa

SEQ ID NO: 533 - DNA, 28 bp, Artificial Sequence
  Description of Artificial Sequence: Synthetic probe
  5' amino modifier C6
cccaacgagtctcttgagaggaaactaa

SEQ ID NO: 534 - DNA, 28 bp, Artificial Sequence
  Description of Artificial Sequence: Synthetic probe
  5' amino modifier C6
cccaacgtagtgagtagacgtacaccaa

SEQ ID NO: 535 - DNA, 28 bp, Artificial Sequence
  Description of Artificial Sequence: Synthetic probe
  5' amino modifier C6
cccaaaaagcttgttaccttctgcagaa

SEQ ID NO: 536 - DNA, 28 bp, Artificial Sequence
  Description of Artificial Sequence: Synthetic probe
  5' amino modifier C6
cccaaactttgtactggagtagccaaaa

SEQ ID NO: 537 - DNA, 28 bp, Artificial Sequence
  Description of Artificial Sequence: Synthetic probe
  5' amino modifier C6
cccaagcttacctcttaagtgcaagaaa

SEQ ID NO: 538 - DNA, 28 bp, Artificial Sequence
  Description of Artificial Sequence: Synthetic probe
  5' amino modifier C6
cccaagaacctcttaaagctaagcgaaa

SEQ ID NO: 539 - DNA, 28 bp, Artificial Sequence
  Description of Artificial Sequence: Synthetic probe
  5' amino modifier C6
cccaagacctaaacaagcttgagtcgaa

SEQ ID NO: 540 - DNA, 28 bp, Artificial Sequence
  Description of Artificial Sequence: Synthetic probe
  5' amino modifier C6
cccaatttgcataggttcttccaacgaa

SEQ ID NO: 541 - DNA, 28 bp, Artificial Sequence
  Description of Artificial Sequence: Synthetic probe
  5' amino modifier C6
cccaagcaagttgcattcctctcatgaa

SEQ ID NO: 542 - DNA, 28 bp, Artificial Sequence
  Description of Artificial Sequence: Synthetic probe
  5' amino modifier C6
cccaatcggtacacgacatacatgagaa

SEQ ID NO: 543 - DNA, 28 bp, Artificial Sequence
  Description of Artificial Sequence: Synthetic probe
  5' amino modifier C6
cccaaacctctgtttctgagtcgaagaa

SEQ ID NO: 544 - DNA, 28 bp, Artificial Sequence
  Description of Artificial Sequence: Synthetic probe
  5' amino modifier C6
cccaaacacgtgttggctagtctaaaaa

SEQ ID NO: 545 - DNA, 28 bp, Artificial Sequence
  Description of Artificial Sequence: Synthetic probe
  5' amino modifier C6
cccaacggtttaagcctttcaccatgaa

SEQ ID NO: 546 - DNA, 28 bp, Artificial Sequence
  Description of Artificial Sequence: Synthetic probe
  5' amino modifier C6
cccaacggttcatggactaactgaggaa

SEQ ID NO: 547 - DNA, 28 bp, Artificial Sequence
  Description of Artificial Sequence: Synthetic probe
  5' amino modifier C6
cccaaaccgttcagtttcacatgggaaa

SEQ ID NO: 548 - DNA, 28 bp, Artificial Sequence
  Description of Artificial Sequence: Synthetic probe
  5' amino modifier C6
cccaagacctctccacttgactgtagaa

SEQ ID NO: 549 - DNA, 28 bp, Artificial Sequence
  Description of Artificial Sequence: Synthetic probe
  5' amino modifier C6
cccaagtctttacctcagtgtagcagaa

SEQ ID NO: 550 - DNA, 28 bp, Artificial Sequence
  Description of Artificial Sequence: Synthetic probe
  5' amino modifier C6
cccaaacagctgagtccttccataagaa

SEQ ID NO: 551 - DNA, 28 bp, Artificial Sequence
  Description of Artificial Sequence: Synthetic probe
  5' amino modifier C6
cccaaaactgtcattgccttcctaggaa

SEQ ID NO: 552 - DNA, 28 bp, Artificial Sequence
  Description of Artificial Sequence: Synthetic probe
  5' amino modifier C6
cccaagtccattcattcgttcgaaggaa

SEQ ID NO: 553 - DNA, 28 bp, Artificial Sequence
  Description of Artificial Sequence: Synthetic probe
  5' amino modifier C6
cccaagtcacctcttggtagtaaggcaa

SEQ ID NO: 554 - DNA, 28 bp, Artificial Sequence
  Description of Artificial Sequence: Synthetic probe
  5' amino modifier C6
cccaaccatcagctttagttggtgacaa

SEQ ID NO: 555 - DNA, 28 bp, Artificial Sequence
  Description of Artificial Sequence: Synthetic probe
  5' amino modifier C6
cccaagttacctgactccactggacaaa

SEQ ID NO: 556 - DNA, 28 bp, Artificial Sequence
  Description of Artificial Sequence: Synthetic probe
  5' amino modifier C6
cccaaagttggcatctttgtcgtcaaaa

SEQ ID NO: 557 - DNA, 28 bp, Artificial Sequence
  Description of Artificial Sequence: Synthetic probe
  5' amino modifier C6
cccaaacgttgtgtctttaacatccgaa

SEQ ID NO: 558 - DNA, 28 bp, Artificial Sequence
  Description of Artificial Sequence: Synthetic probe
  5' amino modifier C6
cccaacagtttggctttgacatcacgaa

SEQ ID NO: 559 - DNA, 28 bp, Artificial Sequence
  Description of Artificial Sequence: Synthetic probe
  5' amino modifier C6
cccaaacggtttgcaactcattcttgaa

SEQ ID NO: 560 - DNA, 28 bp, Artificial Sequence
  Description of Artificial Sequence: Synthetic probe
  5' amino modifier C6
cccaagacgactgtttacttcctcagaa

SEQ ID NO: 561 - DNA, 28 bp, Artificial Sequence
  Description of Artificial Sequence: Synthetic probe
  5' amino modifier C6
cccaaggactccatttcgacttcgacaa

SEQ ID NO: 562 - DNA, 28 bp, Artificial Sequence
  Description of Artificial Sequence: Synthetic probe
  5' amino modifier C6
cccaaatcaagtctagacagaaggctaa

SEQ ID NO: 563 - DNA, 28 bp, Artificial Sequence
  Description of Artificial Sequence: Synthetic probe
  5' amino modifier C6
cccaagtcgtcatcagcaagaaacctaa

SEQ ID NO: 564 - DNA, 28 bp, Artificial Sequence
  Description of Artificial Sequence: Synthetic probe
  5' amino modifier C6
cccaatcgtgtacatggaaagcacataa

SEQ ID NO: 565 - DNA, 28 bp, Artificial Sequence
  Description of Artificial Sequence: Synthetic probe
  5' amino modifier C6
cccaactttgaagcatggagaacactaa

SEQ ID NO: 566 - DNA, 28 bp, Artificial Sequence
  Description of Artificial Sequence: Synthetic probe
  5' amino modifier C6
cccaaaagtcctctgtttagttagcgaa

SEQ ID NO: 567 - DNA, 28 bp, Artificial Sequence
  Description of Artificial Sequence: Synthetic probe
  5' amino modifier C6
cccaagtaaccaaaccatgctagtcgaa

SEQ ID NO: 568 - DNA, 28 bp, Artificial Sequence
  Description of Artificial Sequence: Synthetic probe
  5' amino modifier C6
cccaaggacattgactcaccatcagcaa

SEQ ID NO: 569 - DNA, 28 bp, Artificial Sequence
  Description of Artificial Sequence: Synthetic probe
  5' amino modifier C6
cccaatgggtactgcatacaccatagaa

SEQ ID NO: 570 - DNA, 28 bp, Artificial Sequence
  Description of Artificial Sequence: Synthetic probe
  5' amino modifier C6
cccaaagaactcgtcttcatttacggaa

SEQ ID NO: 571 - DNA, 28 bp, Artificial Sequence
  Description of Artificial Sequence: Synthetic probe
  5' amino modifier C6
cccaaaggtctttgtcctagtacgagaa

SEQ ID NO: 572 - DNA, 28 bp, Artificial Sequence
  Description of Artificial Sequence: Synthetic probe
  5' amino modifier C6
cccaacatggttaaggtcaactcgagaa

SEQ ID NO: 573 - DNA, 28 bp, Artificial Sequence
  Description of Artificial Sequence: Synthetic probe
  5' amino modifier C6
cccaagcttgtaacgacttactctcgaa

SEQ ID NO: 574 - DNA, 28 bp, Artificial Sequence
  Description of Artificial Sequence: Synthetic probe
  5' amino modifier C6
cccaagaccactctcctagcatttggaa

SEQ ID NO: 575 - DNA, 28 bp, Artificial Sequence
  Description of Artificial Sequence: Synthetic probe
  5' amino modifier C6
cccaagtccattcccattggtagcagaa

SEQ ID NO: 576 - DNA, 28 bp, Artificial Sequence
  Description of Artificial Sequence: Synthetic probe
  5' amino modifier C6
cccaacactctgtgtcgtacatagggaa

SEQ ID NO: 577 - DNA, 28 bp, Artificial Sequence
  Description of Artificial Sequence: Synthetic probe
  5' amino modifier C6
cccaaacttgtgtggaaaccgtacccaa

SEQ ID NO: 578 - DNA, 28 bp, Artificial Sequence
  Description of Artificial Sequence: Synthetic probe
  5' amino modifier C6
cccaaatgccttggtgtcatacaggaaa

SEQ ID NO: 579 - DNA, 28 bp, Artificial Sequence
  Description of Artificial Sequence: Synthetic probe
  5' amino modifier C6
cccaatcggaagtcagactagaaactaa

SEQ ID NO: 580 - DNA, 28 bp, Artificial Sequence
  Description of Artificial Sequence: Synthetic probe
  5' amino modifier C6
cccaaccagtaccagaggtgaagtctaa

SEQ ID NO: 581 - DNA, 28 bp, Artificial Sequence
  Description of Artificial Sequence: Synthetic probe
  5' amino modifier C6
cccaacataaagggaaactgagctctaa

SEQ ID NO: 582 - DNA, 28 bp, Artificial Sequence
  Description of Artificial Sequence: Synthetic probe
  5' amino modifier C6
cccaactaagaggagaactccagttgaa

SEQ ID NO: 583 - DNA, 28 bp, Artificial Sequence
  Description of Artificial Sequence: Synthetic probe
  5' amino modifier C6
cccaactaggaagtttactccactcgaa

SEQ ID NO: 584 - DNA, 28 bp, Artificial Sequence
  Description of Artificial Sequence: Synthetic probe
  5' amino modifier C6
cccaacaacgtctgctaaagtaggtcaa

SEQ ID NO: 585 - DNA, 28 bp, Artificial Sequence
  Description of Artificial Sequence: Synthetic probe
  5' amino modifier C6
cccaacgtcatcaacatagtaggctaaa

SEQ ID NO: 586 - DNA, 28 bp, Artificial Sequence
  Description of Artificial Sequence: Synthetic probe
  5' amino modifier C6
cccaaatcgtcactagagagagaactaa

SEQ ID NO: 587 - DNA, 28 bp, Artificial Sequence
  Description of Artificial Sequence: Synthetic probe
  5' amino modifier C6
cccaacttgtcacatgaaggagacctaa

SEQ ID NO: 588 - DNA, 28 bp, Artificial Sequence
  Description of Artificial Sequence: Synthetic probe
  5' amino modifier C6
cccaaggagactctagaaacttccgaaa

SEQ ID NO: 589 - DNA, 28 bp, Artificial Sequence
  Description of Artificial Sequence: Synthetic probe
  5' amino modifier C6
cccaagagttacgcttctacttccagaa

SEQ ID NO: 590 - DNA, 28 bp, Artificial Sequence
  Description of Artificial Sequence: Synthetic probe
  5' amino modifier C6
cccaaaccagtccttaagggtaggtcaa

SEQ ID NO: 591 - DNA, 28 bp, Artificial Sequence
  Description of Artificial Sequence: Synthetic probe
  5' amino modifier C6
cccaaaagcctagaacattacatcggaa

SEQ ID NO: 592 - DNA, 28 bp, Artificial Sequence
  Description of Artificial Sequence: Synthetic probe
  5' amino modifier C6
cccaagctgaaagcactccatcattgaa

SEQ ID NO: 593 - DNA, 28 bp, Artificial Sequence
  Description of Artificial Sequence: Synthetic probe
  5' amino modifier C6
cccaatcagtgtgactccatccctagaa

SEQ ID NO: 594 - DNA, 28 bp, Artificial Sequence
  Description of Artificial Sequence: Synthetic probe
  5' amino modifier C6
cccaagctacttaactctgtttcggaaa

SEQ ID NO: 595 - DNA, 28 bp, Artificial Sequence
  Description of Artificial Sequence: Synthetic probe
  5' amino modifier C6
cccaaatgctttcactggtctagggaaa

SEQ ID NO: 596 - DNA, 28 bp, Artificial Sequence
  Description of Artificial Sequence: Synthetic probe
  5' amino modifier C6
cccaacagttgttcgttcatgaccagaa

SEQ ID NO: 597 - DNA, 28 bp, Artificial Sequence
  Description of Artificial Sequence: Synthetic probe
  5' amino modifier C6
cccaatcacgaaacgactacttagggaa

SEQ ID NO: 598 - DNA, 28 bp, Artificial Sequence
  Description of Artificial Sequence: Synthetic probe
  5' amino modifier C6
cccaacattgtttggttcatcaagcgaa

SEQ ID NO: 599 - DNA, 28 bp, Artificial Sequence
  Description of Artificial Sequence: Synthetic probe
  5' amino modifier C6
cccaaattcttgtggtacaacatgcgaa

SEQ ID NO: 600 - DNA, 28 bp, Artificial Sequence
  Description of Artificial Sequence: Synthetic probe
  5' amino modifier C6
cccaacctgaccaacggttcatttgtaa

SEQ ID NO: 601 - DNA, 28 bp, Artificial Sequence
  Description of Artificial Sequence: Synthetic probe
  5' amino modifier C6
cccaagaccattacgtcttgccttgaaa

SEQ ID NO: 602 - DNA, 28 bp, Artificial Sequence
  Description of Artificial Sequence: Synthetic probe
  5' amino modifier C6
cccaagccatacctcattgagctttgaa

SEQ ID NO: 603 - DNA, 28 bp, Artificial Sequence
  Description of Artificial Sequence: Synthetic probe
  5' amino modifier C6
cccaaaggactcttccgtaacctgtcaa

SEQ ID NO: 604 - DNA, 28 bp, Artificial Sequence
  Description of Artificial Sequence: Synthetic probe
  5' amino modifier C6
cccaaggagtgcatttcgtaacctgaaa

SEQ ID NO: 605 - DNA, 28 bp, Artificial Sequence
  Description of Artificial Sequence: Synthetic probe
  5' amino modifier C6
cccaatcacaagcgaaagtagtgtctaa

SEQ ID NO: 606 - DNA, 28 bp, Artificial Sequence
  Description of Artificial Sequence: Synthetic probe
  5' amino modifier C6
cccaatcgaagagacgacttgagttcaa

SEQ ID NO: 607 - DNA, 28 bp, Artificial Sequence
  Description of Artificial Sequence: Synthetic probe
  5' amino modifier C6
cccaaatggctttggtacaactgacgaa

SEQ ID NO: 608 - DNA, 28 bp, Artificial Sequence
  Description of Artificial Sequence: Synthetic probe
  5' amino modifier C6
cccaagagacgttggaacacctactgaa

SEQ ID NO: 609 - DNA, 28 bp, Artificial Sequence
  Description of Artificial Sequence: Synthetic probe
  5' amino modifier C6
cccaagaaagctgttcaaacctcacgaa

SEQ ID NO: 610 - DNA, 28 bp, Artificial Sequence
  Description of Artificial Sequence: Synthetic probe
  5' amino modifier C6
cccaagtgagtcttcgaaacttcggaaa

SEQ ID NO: 611 - DNA, 28 bp, Artificial Sequence
  Description of Artificial Sequence: Synthetic probe
  5' amino modifier C6
cccaaccagtgttaacggaacttgggaa

SEQ ID NO: 612 - DNA, 28 bp, Artificial Sequence
  Description of Artificial Sequence: Synthetic probe
  5' amino modifier C6
cccaacaggtgtacttggtactacggaa

SEQ ID NO: 613 - DNA, 28 bp, Artificial Sequence
  Description of Artificial Sequence: Synthetic probe
  5' amino modifier C6
cccaagtaccatccttacgtagcttgaa

SEQ ID NO: 614 - DNA, 28 bp, Artificial Sequence
  Description of Artificial Sequence: Synthetic probe
  5' amino modifier C6
cccaagctacttccactaggtacaggaa

SEQ ID NO: 615 - DNA, 28 bp, Artificial Sequence
  Description of Artificial Sequence: Synthetic probe
  5' amino modifier C6
cccaagtacctcaacaagtcaaggctaa

SEQ ID NO: 616 - DNA, 28 bp, Artificial Sequence
  Description of Artificial Sequence: Synthetic probe
  5' amino modifier C6
cccaagtacccaagagactaagcttgaa

SEQ ID NO: 617 - DNA, 28 bp, Artificial Sequence
  Description of Artificial Sequence: Synthetic probe
  5' amino modifier C6
cccaatgaaccaaacactgacctgtgaa

SEQ ID NO: 618 - DNA, 28 bp, Artificial Sequence
  Description of Artificial Sequence: Synthetic probe
  5' amino modifier C6
cccaagtgcacatcgaaccaacttagaa

SEQ ID NO: 619 - DNA, 28 bp, Artificial Sequence
  Description of Artificial Sequence: Synthetic probe
  5' amino modifier C6
cccaatgcttagcgtactaccattagaa

SEQ ID NO: 620 - DNA, 28 bp, Artificial Sequence
  Description of Artificial Sequence: Synthetic probe
  5' amino modifier C6
cccaagtttgacgttcaaccatcacgaa

SEQ ID NO: 621 - DNA, 28 bp, Artificial Sequence
  Description of Artificial Sequence: Synthetic probe
  5' amino modifier C6
cccaatttagcttgtccactcagaggaa

SEQ ID NO: 622 - DNA, 28 bp, Artificial Sequence
  Description of Artificial Sequence: Synthetic probe
  5' amino modifier C6
cccaacgctactttcttagttagagcaa

SEQ ID NO: 623 - DNA, 28 bp, Artificial Sequence
  Description of Artificial Sequence: Synthetic probe
  5' amino modifier C6
cccaaaagcctttccactgttactggaa

SEQ ID NO: 624 - DNA, 28 bp, Artificial Sequence
  Description of Artificial Sequence: Synthetic probe
  5' amino modifier C6
cccaacctgttacctcagacattgggaa

SEQ ID NO: 625 - DNA, 28 bp, Artificial Sequence
  Description of Artificial Sequence: Synthetic probe
  5' amino modifier C6
cccaacgtcatttaggtctctaagggaa

SEQ ID NO: 626 - DNA, 28 bp, Artificial Sequence
  Description of Artificial Sequence: Synthetic probe
  5' amino modifier C6
cccaaacgtcttgggttacactactgaa

SEQ ID NO: 627 - DNA, 28 bp, Artificial Sequence
  Description of Artificial Sequence: Synthetic probe
  5' amino modifier C6
cccaatcacagaaccagtcagctttgaa

SEQ ID NO: 628 - DNA, 28 bp, Artificial Sequence
  Description of Artificial Sequence: Synthetic probe
  5' amino modifier C6
cccaagtggtactctcgtaactccagaa

SEQ ID NO: 629 - DNA, 28 bp, Artificial Sequence
  Description of Artificial Sequence: Synthetic probe
  5' amino modifier C6
cccaagaactcctaccaagactcgtgaa

SEQ ID NO: 630 - DNA, 28 bp, Artificial Sequence
  Description of Artificial Sequence: Synthetic probe
  5' amino modifier C6
cccaatttgacttgaacgcataaccgaa

SEQ ID NO: 631 - DNA, 28 bp, Artificial Sequence
  Description of Artificial Sequence: Synthetic probe
  5' amino modifier C6
cccaattgagacctcacgagaacactaa

SEQ ID NO: 632 - DNA, 28 bp, Artificial Sequence
  Description of Artificial Sequence: Synthetic probe
  5' amino modifier C6
cccaaacaaagtcattgggttcgctaaa

SEQ ID NO: 633 - DNA, 28 bp, Artificial Sequence
  Description of Artificial Sequence: Synthetic probe
  5' amino modifier C6
cccaatcgaacaaacctagagtgctcaa

SEQ ID NO: 634 - DNA, 28 bp, Artificial Sequence
  Description of Artificial Sequence: Synthetic probe
  5' amino modifier C6
cccaaggtcttagctacaacctcatgaa

SEQ ID NO: 635 - DNA, 28 bp, Artificial Sequence
  Description of Artificial Sequence: Synthetic probe
  5' amino modifier C6
cccaagctttgaagccttccaactagaa

SEQ ID NO: 636 - DNA, 28 bp, Artificial Sequence
  Description of Artificial Sequence: Synthetic probe
  5' amino modifier C6
cccaatacaggtgtcacaaactcacgaa

SEQ ID NO: 637 - DNA, 28 bp, Artificial Sequence
  Description of Artificial Sequence: Synthetic probe
  5' amino modifier C6
cccaaccgttcataacaagggaacctaa

SEQ ID NO: 638 - DNA, 28 bp, Artificial Sequence
  Description of Artificial Sequence: Synthetic probe
  5' amino modifier C6
cccaaagtacccaaagcatgtctggaaa

SEQ ID NO: 639 - DNA, 28 bp, Artificial Sequence
  Description of Artificial Sequence: Synthetic probe
  5' amino modifier C6
cccaaatgttctctttacgctagggaaa

SEQ ID NO: 640 - DNA, 28 bp, Artificial Sequence
  Description of Artificial Sequence: Synthetic probe
  5' amino modifier C6
cccaatttgacttcagacgaaagctgaa

SEQ ID NO: 641 - DNA, 28 bp, Artificial Sequence
  Description of Artificial Sequence: Synthetic probe
  5' amino modifier C6
cccaatacagaaacgacatacgcttgaa

SEQ ID NO: 642 - DNA, 28 bp, Artificial Sequence
  Description of Artificial Sequence: Synthetic probe
  5' amino modifier C6
cccaatcaccagaagaactacctgtgaa

SEQ ID NO: 643 - DNA, 28 bp, Artificial Sequence
  Description of Artificial Sequence: Synthetic probe
  5' amino modifier C6
cccaatacgaacgacaggtcatggttaa

SEQ ID NO: 644 - DNA, 28 bp, Artificial Sequence
  Description of Artificial Sequence: Synthetic probe
  5' amino modifier C6
cccaagaactccaaccatgtagtcgtaa

SEQ ID NO: 645 - DNA, 28 bp, Artificial Sequence
  Description of Artificial Sequence: Synthetic probe
  5' amino modifier C6
cccaaattgcgttcttcagtacacgaaa

SEQ ID NO: 646 - DNA, 28 bp, Artificial Sequence
  Description of Artificial Sequence: Synthetic probe
  5' amino modifier C6
cccaaatctgcttcctgtagtacacgaa

SEQ ID NO: 647 - DNA, 28 bp, Artificial Sequence
  Description of Artificial Sequence: Synthetic probe
  5' amino modifier C6
cccaaggtcacttgcaacctagaaccaa

SEQ ID NO: 648 - DNA, 28 bp, Artificial Sequence
  Description of Artificial Sequence: Synthetic probe
  5' amino modifier C6
cccaaggcttagtacgacagtaacccaa

SEQ ID NO: 649 - DNA, 28 bp, Artificial Sequence
  Description of Artificial Sequence: Synthetic probe
  5' amino modifier C6
cccaacaagtgaagtggtctgaccagaa

SEQ ID NO: 650 - DNA, 28 bp, Artificial Sequence
  Description of Artificial Sequence: Synthetic probe
  5' amino modifier C6
cccaacagagtagtgtgactagcctaaa

SEQ ID NO: 651 - DNA, 28 bp, Artificial Sequence
  Description of Artificial Sequence: Synthetic probe
  5' amino modifier C6
cccaatcacaaggagtagcaactttgaa

SEQ ID NO: 652 - DNA, 28 bp, Artificial Sequence
  Description of Artificial Sequence: Synthetic probe
  5' amino modifier C6
cccaacctgtaagtgaaacgactggaaa

SEQ ID NO: 653 - DNA, 28 bp, Artificial Sequence
  Description of Artificial Sequence: Synthetic probe
  5' amino modifier C6
cccaaccctagttgaggacaaactggaa

SEQ ID NO: 654 - DNA, 28 bp, Artificial Sequence
  Description of Artificial Sequence: Synthetic probe
  5' amino modifier C6
cccaaggcatcacacctagcaagtttaa

SEQ ID NO: 655 - DNA, 28 bp, Artificial Sequence
  Description of Artificial Sequence: Synthetic probe
  5' amino modifier C6
cccaagacctaccctacagagcttgtaa

SEQ ID NO: 656 - DNA, 28 bp, Artificial Sequence
  Description of Artificial Sequence: Synthetic probe
  5' amino modifier C6
cccaatttcgtaacaagttggactcgaa

SEQ ID NO: 657 - DNA, 28 bp, Artificial Sequence
  Description of Artificial Sequence: Synthetic probe
  5' amino modifier C6
cccaatcaaagaaacaggttgcactgaa

SEQ ID NO: 658 - DNA, 28 bp, Artificial Sequence
  Description of Artificial Sequence: Synthetic probe
  5' amino modifier C6
cccaacgtcttagagtccttgaacccaa

SEQ ID NO: 659 - DNA, 28 bp, Artificial Sequence
  Description of Artificial Sequence: Synthetic probe
  5' amino modifier C6
cccaatgctgaaacgtttcccttgtaaa

SEQ ID NO: 660 - DNA, 28 bp, Artificial Sequence
  Description of Artificial Sequence: Synthetic probe
  5' amino modifier C6
cccaacaggtttgtttgactcagacgaa

SEQ ID NO: 661 - DNA, 28 bp, Artificial Sequence
  Description of Artificial Sequence: Synthetic probe
  5' amino modifier C6
cccaaccttcgacataaagaaagcgtaa

SEQ ID NO: 662 - DNA, 28 bp, Artificial Sequence
  Description of Artificial Sequence: Synthetic probe
  5' amino modifier C6
cccaatgaaccattagcaagcaaggtaa

SEQ ID NO: 663 - DNA, 28 bp, Artificial Sequence
  Description of Artificial Sequence: Synthetic probe
  5' amino modifier C6
cccaatgaaccttgagcacaaactggaa

SEQ ID NO: 664 - DNA, 28 bp, Artificial Sequence
  Description of Artificial Sequence: Synthetic probe
  5' amino modifier C6
cccaaagggttcttggacagtacctcaa

SEQ ID NO: 665 - DNA, 28 bp, Artificial Sequence
  Description of Artificial Sequence: Synthetic probe
  5' amino modifier C6
cccaactgtaaaggagttcgtaccctaa

SEQ ID NO: 666 - DNA, 28 bp, Artificial Sequence
  Description of Artificial Sequence: Synthetic probe
  5' amino modifier C6
cccaatcgagaaggaagtcacactgtaa

SEQ ID NO: 667 - DNA, 28 bp, Artificial Sequence
  Description of Artificial Sequence: Synthetic probe
  5' amino modifier C6
cccaactaaaggaagtgtcagctgtcaa

SEQ ID NO: 668 - DNA, 28 bp, Artificial Sequence
  Description of Artificial Sequence: Synthetic probe
  5' amino modifier C6
cccaagcacataaggtcaaacgtgtgaa

SEQ ID NO: 669 - DNA, 28 bp, Artificial Sequence
  Description of Artificial Sequence: Synthetic probe
  5' amino modifier C6
cccaacgttgaaggaacattcacaggaa

SEQ ID NO: 670 - DNA, 28 bp, Artificial Sequence
  Description of Artificial Sequence: Synthetic probe
  5' amino modifier C6
cccaatgtgagctgacaaacaacatgaa

SEQ ID NO: 671 - DNA, 28 bp, Artificial Sequence
  Description of Artificial Sequence: Synthetic probe
  5' amino modifier C6
cccaagctactctaacacgactggacaa

SEQ ID NO: 672 - DNA, 28 bp, Artificial Sequence
  Description of Artificial Sequence: Synthetic probe
  5' amino modifier C6
cccaagcctaaccttcaagtgcatgtaa

SEQ ID NO: 673 - DNA, 28 bp, Artificial Sequence
  Description of Artificial Sequence: Synthetic probe
  5' amino modifier C6
cccaagtaaacacctctaggttcggaaa

SEQ ID NO: 674 - DNA, 28 bp, Artificial Sequence
  Description of Artificial Sequence: Synthetic probe
  5' amino modifier C6
cccaagtcttgactctcgactcgaaaaa

SEQ ID NO: 675 - DNA, 28 bp, Artificial Sequence
  Description of Artificial Sequence: Synthetic probe
  5' amino modifier C6
cccaactgcagagtggacttgacaaaaa

SEQ ID NO: 676 - DNA, 28 bp, Artificial Sequence
  Description of Artificial Sequence: Synthetic probe
  5' amino modifier C6
cccaacagctctggtgtacttaagacaa

SEQ ID NO: 677 - DNA, 28 bp, Artificial Sequence
  Description of Artificial Sequence: Synthetic probe
  5' amino modifier C6
cccaatacgagagagacgtttacgacaa

SEQ ID NO: 678 - DNA, 28 bp, Artificial Sequence
  Description of Artificial Sequence: Synthetic probe
  5' amino modifier C6
cccaagtaccctactctcgtcaaggaaa

SEQ ID NO: 679 - DNA, 28 bp, Artificial Sequence
  Description of Artificial Sequence: Synthetic probe
  5' amino modifier C6
cccaataacgacacaactggttaccgaa

SEQ ID NO: 680 - DNA, 28 bp, Artificial Sequence
  Description of Artificial Sequence: Synthetic probe
  5' amino modifier C6
cccaacacgtcataacggtagacctcaa

SEQ ID NO: 681 - DNA, 28 bp, Artificial Sequence
  Description of Artificial Sequence: Synthetic probe
  5' amino modifier C6
cccaatcccaagcaacagtcagtagtaa

SEQ ID NO: 682 - DNA, 28 bp, Artificial Sequence
  Description of Artificial Sequence: Synthetic probe
  5' amino modifier C6
cccaataaacgaacacctgtgagctcaa

SEQ ID NO: 683 - DNA, 28 bp, Artificial Sequence
  Description of Artificial Sequence: Synthetic probe
  5' amino modifier C6
cccaagttaccagactcaacaacggtaa

SEQ ID NO: 684 - DNA, 28 bp, Artificial Sequence
  Description of Artificial Sequence: Synthetic probe
  5' amino modifier C6
cccaagttagcttgaccaaccaacgtaa

SEQ ID NO: 685 - DNA, 28 bp, Artificial Sequence
  Description of Artificial Sequence: Synthetic probe
  5' amino modifier C6
cccaagaccatcactacaggagtcctaa

SEQ ID NO: 686 - DNA, 28 bp, Artificial Sequence
  Description of Artificial Sequence: Synthetic probe
  5' amino modifier C6
cccaagtactcttcttacggtagcagaa

SEQ ID NO: 687 - DNA, 28 bp, Artificial Sequence
  Description of Artificial Sequence: Synthetic probe
  5' amino modifier C6
cccaatttgccatcgacaacgtgaaaaa

SEQ ID NO: 688 - DNA, 28 bp, Artificial Sequence
  Description of Artificial Sequence: Synthetic probe
  5' amino modifier C6
cccaaagtctcttgggtacaacgtgtaa

SEQ ID NO: 689 - DNA, 28 bp, Artificial Sequence
  Description of Artificial Sequence: Synthetic probe
  5' amino modifier C6
cccaatgaccttctcgttacaacggtaa

SEQ ID NO: 690 - DNA, 28 bp, Artificial Sequence
  Description of Artificial Sequence: Synthetic probe
  5' amino modifier C6
cccaataccgttctgttaagaagcgtaa

SEQ ID NO: 691 - DNA, 28 bp, Artificial Sequence
  Description of Artificial Sequence: Synthetic probe
  5' amino modifier C6
cccaaagtccttcctctagttacggaaa

SEQ ID NO: 692 - DNA, 28 bp, Artificial Sequence
  Description of Artificial Sequence: Synthetic probe
  5' amino modifier C6
cccaagccatacaacattggactggtaa

SEQ ID NO: 693 - DNA, 28 bp, Artificial Sequence
  Description of Artificial Sequence: Synthetic probe
  5' amino modifier C6
cccaacctgagaggtaagcttgacttaa

SEQ ID NO: 694 - DNA, 28 bp, Artificial Sequence
  Description of Artificial Sequence: Synthetic probe
  5' amino modifier C6
cccaacacctagtagtcgttggacagaa

SEQ ID NO: 695 - DNA, 28 bp, Artificial Sequence
  Description of Artificial Sequence: Synthetic probe
  5' amino modifier C6
cccaagtacactaaaccgttgcgaaaaa

SEQ ID NO: 696 - DNA, 28 bp, Artificial Sequence
  Description of Artificial Sequence: Synthetic probe
  5' amino modifier C6
cccaaccactggtacggaaagctttaaa

SEQ ID NO: 697 - DNA, 28 bp, Artificial Sequence
  Description of Artificial Sequence: Synthetic probe
  5' amino modifier C6
cccaagaccactctttgaggagtacgaa

SEQ ID NO: 698 - DNA, 28 bp, Artificial Sequence
  Description of Artificial Sequence: Synthetic probe
  5' amino modifier C6
cccaagactgaccttggaaagtaggcaa

SEQ ID NO: 699 - DNA, 28 bp, Artificial Sequence
  Description of Artificial Sequence: Synthetic probe
  5' amino modifier C6
cccaactcacgttacgaaacagaggtaa

SEQ ID NO: 700 - DNA, 28 bp, Artificial Sequence
  Description of Artificial Sequence: Synthetic probe
  5' amino modifier C6
cccaagcgtaacgtcatttactttcgaa

SEQ ID NO: 701 - DNA, 28 bp, Artificial Sequence
  Description of Artificial Sequence: Synthetic probe
  5' amino modifier C6
cccaacgaacgtgtcatttcactttgaa

SEQ ID NO: 702 - DNA, 28 bp, Artificial Sequence
  Description of Artificial Sequence: Synthetic probe
  5' amino modifier C6
cccaaatctctggtgtccatccgaacaa

SEQ ID NO: 703 - DNA, 28 bp, Artificial Sequence
  Description of Artificial Sequence: Synthetic probe
  5' amino modifier C6
cccaaagctttggagtctgtgacaacaa

SEQ ID NO: 704 - DNA, 28 bp, Artificial Sequence
  Description of Artificial Sequence: Synthetic probe
  5' amino modifier C6
cccaagggtactaggcttgtgacaacaa

SEQ ID NO: 705 - DNA, 28 bp, Artificial Sequence
  Description of Artificial Sequence: Synthetic probe
  5' amino modifier C6
cccaatagcgaacacctagttacgacaa

SEQ ID NO: 706 - DNA, 28 bp, Artificial Sequence
  Description of Artificial Sequence: Synthetic probe
  5' amino modifier C6
cccaatcacgagtccaagagttacccaa

SEQ ID NO: 707 - DNA, 28 bp, Artificial Sequence
  Description of Artificial Sequence: Synthetic probe
  5' amino modifier C6
cccaatgagaacaaaggctaaccgttaa

SEQ ID NO: 708 - DNA, 28 bp, Artificial Sequence
  Description of Artificial Sequence: Synthetic probe
  5' amino modifier C6
cccaactcgtcatagaacaccaaggtaa

SEQ ID NO: 709 - DNA, 28 bp, Artificial Sequence
  Description of Artificial Sequence: Synthetic probe
  5' amino modifier C6
cccaactccatgcaagtaaagaacgtaa

SEQ ID NO: 710 - DNA, 28 bp, Artificial Sequence
  Description of Artificial Sequence: Synthetic probe
  5' amino modifier C6
cccaaatgtgactaccgaaacgctttaa

SEQ ID NO: 711 - DNA, 28 bp, Artificial Sequence
  Description of Artificial Sequence: Synthetic probe
  5' amino modifier C6
cccaagacaagttgaccaacgcatctaa

SEQ ID NO: 712 - DNA, 28 bp, Artificial Sequence
  Description of Artificial Sequence: Synthetic probe
  5' amino modifier C6
cccaactgcacagtttacaacctaggaa

SEQ ID NO: 713 - DNA, 28 bp, Artificial Sequence
  Description of Artificial Sequence: Synthetic probe
  5' amino modifier C6
cccaagctgactgtcttaacccttagaa

SEQ ID NO: 714 - DNA, 28 bp, Artificial Sequence
  Description of Artificial Sequence: Synthetic probe
  5' amino modifier C6
cccaaggtcaagtcgacaagctaactaa

SEQ ID NO: 715 - DNA, 28 bp, Artificial Sequence
  Description of Artificial Sequence: Synthetic probe
  5' amino modifier C6
cccaacacgtgagttccaaccctaagaa

SEQ ID NO: 716 - DNA, 28 bp, Artificial Sequence
  Description of Artificial Sequence: Synthetic probe
  5' amino modifier C6
cccaagccataaccatcagtctgagtaa

SEQ ID NO: 717 - DNA, 28 bp, Artificial Sequence
  Description of Artificial Sequence: Synthetic probe
  5' amino modifier C6
cccaagtcaacacactcagcagtagtaa

SEQ ID NO: 718 - DNA, 28 bp, Artificial Sequence
  Description of Artificial Sequence: Synthetic probe
  5' amino modifier C6
cccaagtacctactcatgcttgcagtaa

SEQ ID NO: 719 - DNA, 28 bp, Artificial Sequence
  Description of Artificial Sequence: Synthetic probe
  5' amino modifier C6
cccaaatgtacgtaaagcacaagcctaa

SEQ ID NO: 720 - DNA, 28 bp, Artificial Sequence
  Description of Artificial Sequence: Synthetic probe
  5' amino modifier C6
cccaacgtgtaaaggaactaggctacaa

SEQ ID NO: 721 - DNA, 28 bp, Artificial Sequence
  Description of Artificial Sequence: Synthetic probe
  5' amino modifier C6
cccaaggtcactaactcaggaactccaa

SEQ ID NO: 722 - DNA, 28 bp, Artificial Sequence
  Description of Artificial Sequence: Synthetic probe
  5' amino modifier C6
cccaattcgaagtaagcaacaccatgaa

SEQ ID NO: 723 - DNA, 28 bp, Artificial Sequence
  Description of Artificial Sequence: Synthetic probe
  5' amino modifier C6
cccaatcggaagtgtaaactggacacaa

SEQ ID NO: 724 - DNA, 28 bp, Artificial Sequence
  Description of Artificial Sequence: Synthetic probe
  5' amino modifier C6
cccaagactcacaaaccgtacttggtaa

SEQ ID NO: 725 - DNA, 28 bp, Artificial Sequence
  Description of Artificial Sequence: Synthetic probe
  5' amino modifier C6
cccaacattctgcataggagacagtgaa

SEQ ID NO: 726 - DNA, 28 bp, Artificial Sequence
  Description of Artificial Sequence: Synthetic probe
  5' amino modifier C6
cccaaacccatgcacattgagaactgaa

SEQ ID NO: 727 - DNA, 28 bp, Artificial Sequence
  Description of Artificial Sequence: Synthetic probe
  5' amino modifier C6
cccaatggtcaggactaaactaccagaa

SEQ ID NO: 728 - DNA, 28 bp, Artificial Sequence
  Description of Artificial Sequence: Synthetic probe
  5' amino modifier C6
cccaagcttccagaactttacttgggaa

SEQ ID NO: 729 - DNA, 28 bp, Artificial Sequence
  Description of Artificial Sequence: Synthetic probe
  5' amino modifier C6
cccaagttcaactccaacgtcaggacaa

SEQ ID NO: 730 - DNA, 28 bp, Artificial Sequence
  Description of Artificial Sequence: Synthetic probe
  5' amino modifier C6
cccaagttactaccatacgactcgtgaa

SEQ ID NO: 731 - DNA, 28 bp, Artificial Sequence
  Description of Artificial Sequence: Synthetic probe
  5' amino modifier C6
cccaacagacatgcacttaactcaggaa

SEQ ID NO: 732 - DNA, 28 bp, Artificial Sequence
  Description of Artificial Sequence: Synthetic probe
  5' amino modifier C6
cccaacttgaacctagaaagggtagcaa

SEQ ID NO: 733 - DNA, 28 bp, Artificial Sequence
  Description of Artificial Sequence: Synthetic probe
  5' amino modifier C6
cccaagtcctaccttaagagacgagtaa

SEQ ID NO: 734 - DNA, 28 bp, Artificial Sequence
  Description of Artificial Sequence: Synthetic probe
  5' amino modifier C6
cccaacagttagggaagctttgcatcaa

SEQ ID NO: 735 - DNA, 28 bp, Artificial Sequence
  Description of Artificial Sequence: Synthetic probe
  5' amino modifier C6
cccaacgtctagctagaagaagtttcaa

SEQ ID NO: 736 - DNA, 28 bp, Artificial Sequence
  Description of Artificial Sequence: Synthetic probe
  5' amino modifier C6
cccaatttagtcacctctggaaccgtaa

SEQ ID NO: 737 - DNA, 28 bp, Artificial Sequence
  Description of Artificial Sequence: Synthetic probe
  5' amino modifier C6
cccaacagtgaaggaacctttcgtcaaa

SEQ ID NO: 738 - DNA, 28 bp, Artificial Sequence
  Description of Artificial Sequence: Synthetic probe
  5' amino modifier C6
cccaaaggcttcctttcagacagtttaa

SEQ ID NO: 739 - DNA, 28 bp, Artificial Sequence
  Description of Artificial Sequence: Synthetic probe
  5' amino modifier C6
cccaaacggttgttgagtcgaaccataa

SEQ ID NO: 740 - DNA, 28 bp, Artificial Sequence
  Description of Artificial Sequence: Synthetic probe
  5' amino modifier C6
cccaaacctctgagttggctaaacagaa

SEQ ID NO: 741 - DNA, 28 bp, Artificial Sequence
  Description of Artificial Sequence: Synthetic probe
  5' amino modifier C6
cccaagcagttgtaagaccaagacgtaa

SEQ ID NO: 742 - DNA, 28 bp, Artificial Sequence
  Description of Artificial Sequence: Synthetic probe
  5' amino modifier C6
cccaagagagctaccgtttctttgtaaa

SEQ ID NO: 743 - DNA, 28 bp, Artificial Sequence
  Description of Artificial Sequence: Synthetic probe
  5' amino modifier C6
cccaaagggttctccaagtttacaggaa

SEQ ID NO: 744 - DNA, 28 bp, Artificial Sequence
  Description of Artificial Sequence: Synthetic probe
  5' amino modifier C6
cccaacgttagtgtgttcaagcttcaaa

SEQ ID NO: 745 - DNA, 28 bp, Artificial Sequence
  Description of Artificial Sequence: Synthetic probe
  5' amino modifier C6
cccaactcactgcaaaggtaaaggtcaa

SEQ ID NO: 746 - DNA, 28 bp, Artificial Sequence
  Description of Artificial Sequence: Synthetic probe
  5' amino modifier C6
cccaagagctcacaaggtgttaggtcaa

SEQ ID NO: 747 - DNA, 28 bp, Artificial Sequence
  Description of Artificial Sequence: Synthetic probe
  5' amino modifier C6
cccaactgtctactgaaggagtttgcaa

SEQ ID NO: 748 - DNA, 28 bp, Artificial Sequence
  Description of Artificial Sequence: Synthetic probe
  5' amino modifier C6
cccaaagcttcctttactgactagtgaa

SEQ ID NO: 749 - DNA, 28 bp, Artificial Sequence
  Description of Artificial Sequence: Synthetic probe
  5' amino modifier C6
cccaactgctacccttgagtaaagtcaa

SEQ ID NO: 750 - DNA, 28 bp, Artificial Sequence
  Description of Artificial Sequence: Synthetic probe
  5' amino modifier C6
cccaagctcattcccttgaacagagtaa

SEQ ID NO: 751 - DNA, 28 bp, Artificial Sequence
  Description of Artificial Sequence: Synthetic probe
  5' amino modifier C6
cccaagagactgtgcacaacccttagaa

SEQ ID NO: 752 - DNA, 28 bp, Artificial Sequence
  Description of Artificial Sequence: Synthetic probe
  5' amino modifier C6
cccaacggttaacctcaagtgctaaaaa

SEQ ID NO: 753 - DNA, 28 bp, Artificial Sequence
  Description of Artificial Sequence: Synthetic probe
  5' amino modifier C6
cccaaacccttgggtaagctagagacaa

SEQ ID NO: 754 - DNA, 28 bp, Artificial Sequence
  Description of Artificial Sequence: Synthetic probe
  5' amino modifier C6
cccaaattgctcacgttctcatggacaa

SEQ ID NO: 755 - DNA, 28 bp, Artificial Sequence
  Description of Artificial Sequence: Synthetic probe
  5' amino modifier C6
cccaaccctaggaagccatcagtttaaa

SEQ ID NO: 756 - DNA, 28 bp, Artificial Sequence
  Description of Artificial Sequence: Synthetic probe
  5' amino modifier C6
cccaaaccgtttgaaccttctggtcaaa

SEQ ID NO: 757 - DNA, 28 bp, Artificial Sequence
  Description of Artificial Sequence: Synthetic probe
  5' amino modifier C6
cccaatccgaaggagaactttgaccaaa

SEQ ID NO: 758 - DNA, 28 bp, Artificial Sequence
  Description of Artificial Sequence: Synthetic probe
  5' amino modifier C6
cccaattgagtctgaagcaaccaagtaa

SEQ ID NO: 759 - DNA, 28 bp, Artificial Sequence
  Description of Artificial Sequence: Synthetic probe
  5' amino modifier C6
cccaactgtttagagtgacattgcctaa

SEQ ID NO: 760 - DNA, 28 bp, Artificial Sequence
  Description of Artificial Sequence: Synthetic probe
  5' amino modifier C6
cccaatactgttaaggctacaacgctaa

SEQ ID NO: 761 - DNA, 28 bp, Artificial Sequence
  Description of Artificial Sequence: Synthetic probe
  5' amino modifier C6
cccaaatcggttcgttcactactcagaa

SEQ ID NO: 762 - DNA, 28 bp, Artificial Sequence
  Description of Artificial Sequence: Synthetic probe
  5' amino modifier C6
cccaaccaaggttggcttagtagtccaa

SEQ ID NO: 763 - DNA, 28 bp, Artificial Sequence
  Description of Artificial Sequence: Synthetic probe
  5' amino modifier C6
cccaaggctacagactttcccatttgaa

SEQ ID NO: 764 - DNA, 28 bp, Artificial Sequence
  Description of Artificial Sequence: Synthetic probe
  5' amino modifier C6
cccaagaacctcacgtgtgcttgttaaa

SEQ ID NO: 765 - DNA, 28 bp, Artificial Sequence
  Description of Artificial Sequence: Synthetic probe
  5' amino modifier C6
cccaagacatccactcttgtttgacgaa

SEQ ID NO: 766 - DNA, 28 bp, Artificial Sequence
  Description of Artificial Sequence: Synthetic probe
  5' amino modifier C6
cccaaggtacacacctttgccttacgaa

SEQ ID NO: 767 - DNA, 28 bp, Artificial Sequence
  Description of Artificial Sequence: Synthetic probe
  5' amino modifier C6
cccaacgagttggagtaacatacgacaa

SEQ ID NO: 768 - DNA, 28 bp, Artificial Sequence
  Description of Artificial Sequence: Synthetic probe
  5' amino modifier C6
cccaaacggttgtggtaacatcctagaa

SEQ ID NO: 769 - DNA, 28 bp, Artificial Sequence
  Description of Artificial Sequence: Synthetic probe
  5' amino modifier C6
cccaagaccttgactggagaaacggtaa

SEQ ID NO: 770 - DNA, 28 bp, Artificial Sequence
  Description of Artificial Sequence: Synthetic probe
  5' amino modifier C6
cccaagctcactaccattgtcattggaa

SEQ ID NO: 771 - DNA, 28 bp, Artificial Sequence
  Description of Artificial Sequence: Synthetic probe
  5' amino modifier C6
cccaatccgttacgtgaagggtaaacaa

SEQ ID NO: 772 - DNA, 28 bp, Artificial Sequence
  Description of Artificial Sequence: Synthetic probe
  5' amino modifier C6
cccaatacagactgcacactcaggtaaa

SEQ ID NO: 773 - DNA, 28 bp, Artificial Sequence
  Description of Artificial Sequence: Synthetic probe
  5' amino modifier C6
cccaatttacgtagtccaacttgcgaaa

SEQ ID NO: 774 - DNA, 28 bp, Artificial Sequence
  Description of Artificial Sequence: Synthetic probe
  5' amino modifier C6
cccaagaccttactacctgaagcagtaa

SEQ ID NO: 775 - DNA, 28 bp, Artificial Sequence
  Description of Artificial Sequence: Synthetic probe
  5' amino modifier C6
cccaacattgtttctctgacaagctgaa

SEQ ID NO: 776 - DNA, 28 bp, Artificial Sequence
  Description of Artificial Sequence: Synthetic probe
  5' amino modifier C6
cccaacagcagtttagccaagaagtcaa

SEQ ID NO: 777 - DNA, 28 bp, Artificial Sequence
  Description of Artificial Sequence: Synthetic probe
  5' amino modifier C6
cccaagaccttggactctctctaacgaa

SEQ ID NO: 778 - DNA, 28 bp, Artificial Sequence
  Description of Artificial Sequence: Synthetic probe
  5' amino modifier C6
cccaagtactttcttccagtcagagcaa

SEQ ID NO: 779 - DNA, 28 bp, Artificial Sequence
  Description of Artificial Sequence: Synthetic probe
  5' amino modifier C6
cccaatcagacaaccttgttcatcggaa

SEQ ID NO: 780 - DNA, 28 bp, Artificial Sequence
  Description of Artificial Sequence: Synthetic probe
  5' amino modifier C6
cccaatcacctgttgcattcatagggaa

SEQ ID NO: 781 - DNA, 28 bp, Artificial Sequence
  Description of Artificial Sequence: Synthetic probe
  5' amino modifier C6
cccaatttgcagtgaacaccaacagtaa

SEQ ID NO: 782 - DNA, 28 bp, Artificial Sequence
  Description of Artificial Sequence: Synthetic probe
  5' amino modifier C6
cccaagtctgcagtaacacaccaagtaa

SEQ ID NO: 783 - DNA, 28 bp, Artificial Sequence
  Description of Artificial Sequence: Synthetic probe
  5' amino modifier C6
cccaatgtctcagtctccacattaggaa

SEQ ID NO: 784 - DNA, 28 bp, Artificial Sequence
  Description of Artificial Sequence: Synthetic probe
  5' amino modifier C6
cccaagtacaccatttcgcatttcggaa

SEQ ID NO: 785 - DNA, 28 bp, Artificial Sequence
  Description of Artificial Sequence: Synthetic probe
  5' amino modifier C6
cccaagctaccactttagaagtaggcaa

SEQ ID NO: 786 - DNA, 28 bp, Artificial Sequence
  Description of Artificial Sequence: Synthetic probe
  5' amino modifier C6
cccaatcacaaggttaccacaggagtaa

SEQ ID NO: 787 - DNA, 28 bp, Artificial Sequence
  Description of Artificial Sequence: Synthetic probe
  5' amino modifier C6
cccaacaccatggacacttctaagggaa

SEQ ID NO: 788 - DNA, 28 bp, Artificial Sequence
  Description of Artificial Sequence: Synthetic probe
  5' amino modifier C6
cccaacctgaaagagtttcttgcgtaaa

SEQ ID NO: 789 - DNA, 28 bp, Artificial Sequence
  Description of Artificial Sequence: Synthetic probe
  5' amino modifier C6
cccaagagacgtgtcatctcatccagaa

SEQ ID NO: 790 - DNA, 28 bp, Artificial Sequence
  Description of Artificial Sequence: Synthetic probe
  5' amino modifier C6
cccaatagcgtagacaacttcaaagcaa

SEQ ID NO: 791 - DNA, 28 bp, Artificial Sequence
  Description of Artificial Sequence: Synthetic probe
  5' amino modifier C6
cccaaagttctctcgttcatagctgaaa

SEQ ID NO: 792 - DNA, 28 bp, Artificial Sequence
  Description of Artificial Sequence: Synthetic probe
  5' amino modifier C6
cccaaattggtcttctgcataaagcgaa

SEQ ID NO: 793 - DNA, 28 bp, Artificial Sequence
  Description of Artificial Sequence: Synthetic probe
  5' amino modifier C6
cccaatcgaaggagtagtctacctgtaa

SEQ ID NO: 794 - DNA, 28 bp, Artificial Sequence
  Description of Artificial Sequence: Synthetic probe
  5' amino modifier C6
cccaatcaggactacggaaagttcccaa

SEQ ID NO: 795 - DNA, 28 bp, Artificial Sequence
  Description of Artificial Sequence: Synthetic probe
  5' amino modifier C6
cccaaccgtaacatccatgagacgtcaa

SEQ ID NO: 796 - DNA, 28 bp, Artificial Sequence
  Description of Artificial Sequence: Synthetic probe
  5' amino modifier C6
cccaatgcgaaagaggtaccgtttacaa

SEQ ID NO: 797 - DNA, 28 bp, Artificial Sequence
  Description of Artificial Sequence: Synthetic probe
  5' amino modifier C6
cccaagacacatccaactggtgactcaa

SEQ ID NO: 798 - DNA, 28 bp, Artificial Sequence
  Description of Artificial Sequence: Synthetic probe
  5' amino modifier C6
cccaagaccatccttcaagagacgtcaa

SEQ ID NO: 799 - DNA, 28 bp, Artificial Sequence
  Description of Artificial Sequence: Synthetic probe
  5' amino modifier C6
cccaagctctcaagtctaaacagtgcaa

SEQ ID NO: 800 - DNA, 28 bp, Artificial Sequence
  Description of Artificial Sequence: Synthetic probe
  5' amino modifier C6
cccaacaaagtagaaactcgtagctgaa

SEQ ID NO: 801 - DNA, 28 bp, Artificial Sequence
  Description of Artificial Sequence: Synthetic probe
  5' amino modifier C6
cccaaccagagtgtgaacactagggtaa

SEQ ID NO: 802 - DNA, 28 bp, Artificial Sequence
  Description of Artificial Sequence: Synthetic probe
  5' amino modifier C6
cccaacctcatgaagactccaagggtaa

SEQ ID NO: 803 - DNA, 28 bp, Artificial Sequence
  Description of Artificial Sequence: Synthetic probe
  5' amino modifier C6
cccaaacctgtggacactacaccttgaa

SEQ ID NO: 804 - DNA, 28 bp, Artificial Sequence
  Description of Artificial Sequence: Synthetic probe
  5' amino modifier C6
cccaaagttcagagttctctccactgaa

SEQ ID NO: 805 - DNA, 28 bp, Artificial Sequence
  Description of Artificial Sequence: Synthetic probe
  5' amino modifier C6
cccaagctactttcaactgacagtggaa

SEQ ID NO: 806 - DNA, 28 bp, Artificial Sequence
  Description of Artificial Sequence: Synthetic probe
  5' amino modifier C6
cccaagccatcttctactgaacggtaaa

SEQ ID NO: 807 - DNA, 28 bp, Artificial Sequence
  Description of Artificial Sequence: Synthetic probe
  5' amino modifier C6
cccaatgtttcagtccattgaacgctaa

SEQ ID NO: 808 - DNA, 28 bp, Artificial Sequence
  Description of Artificial Sequence: Synthetic probe
  5' amino modifier C6
cccaaattgcttctcacgtcattaggaa

SEQ ID NO: 809 - DNA, 28 bp, Artificial Sequence
  Description of Artificial Sequence: Synthetic probe
  5' amino modifier C6
cccaatgggaactctgaaacatccgaaa

SEQ ID NO: 810 - DNA, 28 bp, Artificial Sequence
  Description of Artificial Sequence: Synthetic probe
  5' amino modifier C6
cccaatcgtagagtcaaaccacaagtaa

SEQ ID NO: 811 - DNA, 28 bp, Artificial Sequence
  Description of Artificial Sequence: Synthetic probe
  5' amino modifier C6
cccaacaggtgtcgtgtgaaacagtcaa

SEQ ID NO: 812 - DNA, 28 bp, Artificial Sequence
  Description of Artificial Sequence: Synthetic probe
  5' amino modifier C6
cccaaggtcattaagccttcgactccaa

SEQ ID NO: 813 - DNA, 28 bp, Artificial Sequence
  Description of Artificial Sequence: Synthetic probe
  5' amino modifier C6
cccaacttgaagtgaaggcaaccatgaa

SEQ ID NO: 814 - DNA, 28 bp, Artificial Sequence
  Description of Artificial Sequence: Synthetic probe
  5' amino modifier C6
cccaacaactaggagtgctctggttaaa

SEQ ID NO: 815 - DNA, 28 bp, Artificial Sequence
  Description of Artificial Sequence: Synthetic probe
  5' amino modifier C6
cccaagaccatagcatccaagtcgtcaa

SEQ ID NO: 816 - DNA, 28 bp, Artificial Sequence
  Description of Artificial Sequence: Synthetic probe
  5' amino modifier C6
cccaatcgagaaacacctgtacaagtaa

SEQ ID NO: 817 - DNA, 28 bp, Artificial Sequence
  Description of Artificial Sequence: Synthetic probe
  5' amino modifier C6
cccaacagtctttaagcagaaggactaa

SEQ ID NO: 818 - DNA, 28 bp, Artificial Sequence
  Description of Artificial Sequence: Synthetic probe
  5' amino modifier C6
cccaacgtcaactacacagaaggtctaa

SEQ ID NO: 819 - DNA, 28 bp, Artificial Sequence
  Description of Artificial Sequence: Synthetic probe
  5' amino modifier C6
cccaagtcgacaacagcattaggtctaa

SEQ ID NO: 820 - DNA, 28 bp, Artificial Sequence
  Description of Artificial Sequence: Synthetic probe
  5' amino modifier C6
cccaattggtcagaactttccttgcaaa

SEQ ID NO: 821 - DNA, 28 bp, Artificial Sequence
  Description of Artificial Sequence: Synthetic probe
  5' amino modifier C6
cccaacctaggtcaagtttaggttgcaa

SEQ ID NO: 822 - DNA, 28 bp, Artificial Sequence
  Description of Artificial Sequence: Synthetic probe
  5' amino modifier C6
cccaagtcatctgcatccacactaggaa

SEQ ID NO: 823 - DNA, 28 bp, Artificial Sequence
  Description of Artificial Sequence: Synthetic probe
  5' amino modifier C6
cccaaatcgcttgaaccataccatggaa

SEQ ID NO: 824 - DNA, 28 bp, Artificial Sequence
  Description of Artificial Sequence: Synthetic probe
  5' amino modifier C6
cccaaatctgaactgaggaacaagctaa

SEQ ID NO: 825 - DNA, 28 bp, Artificial Sequence
  Description of Artificial Sequence: Synthetic probe
  5' amino modifier C6
cccaacgtgagcatcaggaacatttgaa

SEQ ID NO: 826 - DNA, 28 bp, Artificial Sequence
  Description of Artificial Sequence: Synthetic probe
  5' amino modifier C6
cccaatccctagttccagtcatgaggaa

SEQ ID NO: 827 - DNA, 28 bp, Artificial Sequence
  Description of Artificial Sequence: Synthetic probe
  5' amino modifier C6
cccaactcctagtcctgtagtccagaaa

SEQ ID NO: 828 - DNA, 28 bp, Artificial Sequence
  Description of Artificial Sequence: Synthetic probe
  5' amino modifier C6
cccaagagtcaactccatgaaagcctaa

SEQ ID NO: 829 - DNA, 28 bp, Artificial Sequence
  Description of Artificial Sequence: Synthetic probe
  5' amino modifier C6
cccaaggtagtctcagagaacacctgaa

SEQ ID NO: 830 - DNA, 28 bp, Artificial Sequence
  Description of Artificial Sequence: Synthetic probe
  5' amino modifier C6
cccaagctgtaggacataagaaccgtaa

SEQ ID NO: 831 - DNA, 28 bp, Artificial Sequence
  Description of Artificial Sequence: Synthetic probe
  5' amino modifier C6
cccaagtccaactgaaacagagctgtaa

SEQ ID NO: 832 - DNA, 28 bp, Artificial Sequence
  Description of Artificial Sequence: Synthetic probe
  5' amino modifier C6
cccaagtgcaactacaggacagtgtgaa

SEQ ID NO: 833 - DNA, 28 bp, Artificial Sequence
  Description of Artificial Sequence: Synthetic probe
  5' amino modifier C6
cccaatgaaacagacaagtagcgttcaa

SEQ ID NO: 834 - DNA, 28 bp, Artificial Sequence
  Description of Artificial Sequence: Synthetic probe
  5' amino modifier C6
cccaaaaactgtagctttcccttggaaa

SEQ ID NO: 835 - DNA, 28 bp, Artificial Sequence
  Description of Artificial Sequence: Synthetic probe
  5' amino modifier C6
cccaatccgtagagcagtgagtttacaa

SEQ ID NO: 836 - DNA, 28 bp, Artificial Sequence
  Description of Artificial Sequence: Synthetic probe
  5' amino modifier C6
cccaaggttcatgcatcctcttcaagaa

SEQ ID NO: 837 - DNA, 28 bp, Artificial Sequence
  Description of Artificial Sequence: Synthetic probe
  5' amino modifier C6
cccaaacctttgtggagtcaagcatgaa

SEQ ID NO: 838 - DNA, 28 bp, Artificial Sequence
  Description of Artificial Sequence: Synthetic probe
  5' amino modifier C6
cccaaacctttgtgagcagagcatttaa

SEQ ID NO: 839 - DNA, 28 bp, Artificial Sequence
  Description of Artificial Sequence: Synthetic probe
  5' amino modifier C6
cccaaactgtttcccttagagcagtcaa

SEQ ID NO: 840 - DNA, 28 bp, Artificial Sequence
  Description of Artificial Sequence: Synthetic probe
  5' amino modifier C6
cccaagctgtaggagttacatctctgaa

SEQ ID NO: 841 - DNA, 28 bp, Artificial Sequence
  Description of Artificial Sequence: Synthetic probe
  5' amino modifier C6
cccaagtggacactccagaactctgtaa

SEQ ID NO: 842 - DNA, 28 bp, Artificial Sequence
  Description of Artificial Sequence: Synthetic probe
  5' amino modifier C6
cccaacgtcatctgacagaacagactaa

SEQ ID NO: 843 - DNA, 28 bp, Artificial Sequence
  Description of Artificial Sequence: Synthetic probe
  5' amino modifier C6
cccaagtccaacgaagcatgacacttaa

SEQ ID NO: 844 - DNA, 28 bp, Artificial Sequence
  Description of Artificial Sequence: Synthetic probe
  5' amino modifier C6
cccaaagcctaaagcctttgggttacaa

SEQ ID NO: 845 - DNA, 28 bp, Artificial Sequence
  Description of Artificial Sequence: Synthetic probe
  5' amino modifier C6
cccaaccgttcaaacgactaagagtcaa

SEQ ID NO: 846 - DNA, 28 bp, Artificial Sequence
  Description of Artificial Sequence: Synthetic probe
  5' amino modifier C6
cccaatcggaacacctttggtttccaaa

SEQ ID NO: 847 - DNA, 28 bp, Artificial Sequence
  Description of Artificial Sequence: Synthetic probe
  5' amino modifier C6
cccaatgaccatcatgtttggcttcaaa

SEQ ID NO: 848 - DNA, 28 bp, Artificial Sequence
  Description of Artificial Sequence: Synthetic probe
  5' amino modifier C6
cccaagaccatgagctctcttgttcaaa

SEQ ID NO: 849 - DNA, 28 bp, Artificial Sequence
  Description of Artificial Sequence: Synthetic probe
  5' amino modifier C6
cccaactaggtgaagtgacagcatccaa

SEQ ID NO: 850 - DNA, 28 bp, Artificial Sequence
  Description of Artificial Sequence: Synthetic probe
  5' amino modifier C6
cccaacaagttaggagactgactgcaaa

SEQ ID NO: 851 - DNA, 28 bp, Artificial Sequence
  Description of Artificial Sequence: Synthetic probe
  5' amino modifier C6
cccaatcagcacacgagttctagtaaaa

SEQ ID NO: 852 - DNA, 28 bp, Artificial Sequence
  Description of Artificial Sequence: Synthetic probe
  5' amino modifier C6
cccaaacgtcacctaggttgggttacaa

SEQ ID NO: 853 - DNA, 28 bp, Artificial Sequence
  Description of Artificial Sequence: Synthetic probe
  5' amino modifier C6
cccaaaccttgtctcttagccatggaaa

SEQ ID NO: 854 - DNA, 28 bp, Artificial Sequence
  Description of Artificial Sequence: Synthetic probe
  5' amino modifier C6
cccaaaccttgttactgtgctagagcaa

SEQ ID NO: 855 - DNA, 28 bp, Artificial Sequence
  Description of Artificial Sequence: Synthetic probe
  5' amino modifier C6
cccaaacagagtgcttccaacttctgaa

SEQ ID NO: 856 - DNA, 28 bp, Artificial Sequence
  Description of Artificial Sequence: Synthetic probe
  5' amino modifier C6
cccaatcgttcacgaagtagggttacaa

SEQ ID NO: 857 - DNA, 28 bp, Artificial Sequence
  Description of Artificial Sequence: Synthetic probe
  5' amino modifier C6
cccaaaaacatgttccgtagttgccaaa

SEQ ID NO: 858 - DNA, 28 bp, Artificial Sequence
  Description of Artificial Sequence: Synthetic probe
  5' amino modifier C6
cccaatgaccacaacatagcatgtcgaa

SEQ ID NO: 859 - DNA, 28 bp, Artificial Sequence
  Description of Artificial Sequence: Synthetic probe
  5' amino modifier C6
cccaagcataaacactctggacaggtaa

SEQ ID NO: 860 - DNA, 28 bp, Artificial Sequence
  Description of Artificial Sequence: Synthetic probe
  5' amino modifier C6
cccaagctaacaaccatcgagagtctaa

SEQ ID NO: 861 - DNA, 28 bp, Artificial Sequence
  Description of Artificial Sequence: Synthetic probe
  5' amino modifier C6
cccaagtgaaactcacacgagactctaa

SEQ ID NO: 862 - DNA, 28 bp, Artificial Sequence
  Description of Artificial Sequence: Synthetic probe
  5' amino modifier C6
cccaagtaacaaacccatgagctgtgaa

SEQ ID NO: 863 - DNA, 28 bp, Artificial Sequence
  Description of Artificial Sequence: Synthetic probe
  5' amino modifier C6
cccaagtcgacatcacagtcaaggtgaa

SEQ ID NO: 864 - DNA, 28 bp, Artificial Sequence
  Description of Artificial Sequence: Synthetic probe
  5' amino modifier C6
cccaagaactctctctgcacattgtgaa

SEQ ID NO: 865 - DNA, 28 bp, Artificial Sequence
  Description of Artificial Sequence: Synthetic probe
  5' amino modifier C6
cccaactgcacacatggtttctttgaaa

SEQ ID NO: 866 - DNA, 28 bp, Artificial Sequence
  Description of Artificial Sequence: Synthetic probe
  5' amino modifier C6
cccaataaagcactttgagagtaccgaa

SEQ ID NO: 867 - DNA, 28 bp, Artificial Sequence
  Description of Artificial Sequence: Synthetic probe
  5' amino modifier C6
cccaaatcgcttgtttaacctactggaa

SEQ ID NO: 868 - DNA, 28 bp, Artificial Sequence
  Description of Artificial Sequence: Synthetic probe
  5' amino modifier C6
cccaacgttgagtttaagctaccagaaa

SEQ ID NO: 869 - DNA, 28 bp, Artificial Sequence
  Description of Artificial Sequence: Synthetic probe
  5' amino modifier C6
cccaagtttcactacacgacttcgagaa

SEQ ID NO: 870 - DNA, 28 bp, Artificial Sequence
  Description of Artificial Sequence: Synthetic probe
  5' amino modifier C6
cccaatggagacagtcttccctttgaaa

SEQ ID NO: 871 - DNA, 28 bp, Artificial Sequence
  Description of Artificial Sequence: Synthetic probe
  5' amino modifier C6
cccaagtttcactgcacttcaaggtgaa

SEQ ID NO: 872 - DNA, 28 bp, Artificial Sequence
  Description of Artificial Sequence: Synthetic probe
  5' amino modifier C6
cccaaccagtctggttctactacacgaa

SEQ ID NO: 873 - DNA, 28 bp, Artificial Sequence
  Description of Artificial Sequence: Synthetic probe
  5' amino modifier C6
cccaaattctcgttctcagagtcaggaa

SEQ ID NO: 874 - DNA, 28 bp, Artificial Sequence
  Description of Artificial Sequence: Synthetic probe
  5' amino modifier C6
cccaagttaccaacacctgagaagctaa

SEQ ID NO: 875 - DNA, 28 bp, Artificial Sequence
  Description of Artificial Sequence: Synthetic probe
  5' amino modifier C6
cccaaactactgtcaaaggagtaggcaa

SEQ ID NO: 876 - DNA, 28 bp, Artificial Sequence
  Description of Artificial Sequence: Synthetic probe
  5' amino modifier C6
cccaagttcccaagacctacaagctgaa

SEQ ID NO: 877 - DNA, 28 bp, Artificial Sequence
  Description of Artificial Sequence: Synthetic probe
  5' amino modifier C6
cccaatttagcctaacagcaacaggtaa

SEQ ID NO: 878 - DNA, 28 bp, Artificial Sequence
  Description of Artificial Sequence: Synthetic probe
  5' amino modifier C6
cccaaatctgttctctgcaaagtcgtaa

SEQ ID NO: 879 - DNA, 28 bp, Artificial Sequence
  Description of Artificial Sequence: Synthetic probe
  5' amino modifier C6
cccaaagtccttgtctcaaactcaggaa

SEQ ID NO: 880 - DNA, 28 bp, Artificial Sequence
  Description of Artificial Sequence: Synthetic probe
  5' amino modifier C6
cccaaatcttgtgtgtcgaagcaactaa

SEQ ID NO: 881 - DNA, 28 bp, Artificial Sequence
  Description of Artificial Sequence: Synthetic probe
  5' amino modifier C6
cccaagtgcaactggagacagactttaa

SEQ ID NO: 882 - DNA, 28 bp, Artificial Sequence
  Description of Artificial Sequence: Synthetic probe
  5' amino modifier C6
cccaaactgtcttgttcgaacagcataa

SEQ ID NO: 883 - DNA, 28 bp, Artificial Sequence
  Description of Artificial Sequence: Synthetic probe
  5' amino modifier C6
cccaatttgtacatcgcttcatcggaaa

SEQ ID NO: 884 - DNA, 28 bp, Artificial Sequence
  Description of Artificial Sequence: Synthetic probe
  5' amino modifier C6
cccaatacagaaggagtacctgacctaa

SEQ ID NO: 885 - DNA, 28 bp, Artificial Sequence
  Description of Artificial Sequence: Synthetic probe
  5' amino modifier C6
cccaatcgcaaagaagtaccagtttcaa

SEQ ID NO: 886 - DNA, 28 bp, Artificial Sequence
  Description of Artificial Sequence: Synthetic probe
  5' amino modifier C6
cccaactggtagacatgcatagaagcaa

SEQ ID NO: 887 - DNA, 28 bp, Artificial Sequence
  Description of Artificial Sequence: Synthetic probe
  5' amino modifier C6
cccaagagaactaccgttgtgaaggcaa

SEQ ID NO: 888 - DNA, 28 bp, Artificial Sequence
  Description of Artificial Sequence: Synthetic probe
  5' amino modifier C6
cccaatttcgagagtcacatcaacagaa

SEQ ID NO: 889 - DNA, 28 bp, Artificial Sequence
  Description of Artificial Sequence: Synthetic probe
  5' amino modifier C6
cccaacggtaaggctacctctttgtaaa

SEQ ID NO: 890 - DNA, 28 bp, Artificial Sequence
  Description of Artificial Sequence: Synthetic probe
  5' amino modifier C6
cccaactacgctactaaagtaaaggcaa

SEQ ID NO: 891 - DNA, 28 bp, Artificial Sequence
  Description of Artificial Sequence: Synthetic probe
  5' amino modifier C6
cccaacgtgagttcgttaactaccagaa

SEQ ID NO: 892 - DNA, 28 bp, Artificial Sequence
  Description of Artificial Sequence: Synthetic probe
  5' amino modifier C6
cccaatggtctagcattcaactaccgaa

SEQ ID NO: 893 - DNA, 28 bp, Artificial Sequence
  Description of Artificial Sequence: Synthetic probe
  5' amino modifier C6
cccaatgtttcagacctgactacctgaa

SEQ ID NO: 894 - DNA, 28 bp, Artificial Sequence
  Description of Artificial Sequence: Synthetic probe
  5' amino modifier C6
cccaataacagaacccatgctcaggtaa

SEQ ID NO: 895 - DNA, 28 bp, Artificial Sequence
  Description of Artificial Sequence: Synthetic probe
  5' amino modifier C6
cccaaacacgttgcactttactttggaa

SEQ ID NO: 896 - DNA, 28 bp, Artificial Sequence
  Description of Artificial Sequence: Synthetic probe
  5' amino modifier C6
cccaatgctgacgtacacaaacaagtaa

SEQ ID NO: 897 - DNA, 28 bp, Artificial Sequence
  Description of Artificial Sequence: Synthetic probe
  5' amino modifier C6
cccaaagctgttgctgttaaaccgtaaa

SEQ ID NO: 898 - DNA, 28 bp, Artificial Sequence
  Description of Artificial Sequence: Synthetic probe
  5' amino modifier C6
cccaacatgttgtggtagctaccgaaaa

SEQ ID NO: 899 - DNA, 28 bp, Artificial Sequence
  Description of Artificial Sequence: Synthetic probe
  5' amino modifier C6
cccaaatctctgtggtagcataacggaa

SEQ ID NO: 900 - DNA, 28 bp, Artificial Sequence
  Description of Artificial Sequence: Synthetic probe
  5' amino modifier C6
cccaagagctctcgtgttactaaagtaa

SEQ ID NO: 901 - DNA, 28 bp, Artificial Sequence
  Description of Artificial Sequence: Synthetic probe
  5' amino modifier C6
cccaaagccttggttgtcagtcttaaaa

SEQ ID NO: 902 - DNA, 28 bp, Artificial Sequence
  Description of Artificial Sequence: Synthetic probe
  5' amino modifier C6
cccaagtacctctactctgactcaggaa

SEQ ID NO: 903 - DNA, 28 bp, Artificial Sequence
  Description of Artificial Sequence: Synthetic probe
  5' amino modifier C6
cccaaggcatacaactctgacctgtcaa

SEQ ID NO: 904 - DNA, 28 bp, Artificial Sequence
  Description of Artificial Sequence: Synthetic probe
  5' amino modifier C6
cccaaccagtaaaccagtgacttgccaa

SEQ ID NO: 905 - DNA, 28 bp, Artificial Sequence
  Description of Artificial Sequence: Synthetic probe
  5' amino modifier C6
cccaagactccttggttcaacggtaaaa

SEQ ID NO: 906 - DNA, 28 bp, Artificial Sequence
  Description of Artificial Sequence: Synthetic probe
  5' amino modifier C6
cccaacttaggtaggtagcacactgaaa

SEQ ID NO: 907 - DNA, 28 bp, Artificial Sequence
  Description of Artificial Sequence: Synthetic probe
  5' amino modifier C6
cccaaagtccagagcacatttcatagaa

SEQ ID NO: 908 - DNA, 28 bp, Artificial Sequence
  Description of Artificial Sequence: Synthetic probe
  5' amino modifier C6
cccaaggctacatgtcacctaaccagaa

SEQ ID NO: 909 - DNA, 28 bp, Artificial Sequence
  Description of Artificial Sequence: Synthetic probe
  5' amino modifier C6
cccaatgtccatgactttcctaacggaa

SEQ ID NO: 910 - DNA, 28 bp, Artificial Sequence
  Description of Artificial Sequence: Synthetic probe
  5' amino modifier C6
cccaagcacatggttccacataaacgaa

SEQ ID NO: 911 - DNA, 28 bp, Artificial Sequence
  Description of Artificial Sequence: Synthetic probe
  5' amino modifier C6
cccaagccatgttgcacactacaaagaa

SEQ ID NO: 912 - DNA, 28 bp, Artificial Sequence
  Description of Artificial Sequence: Synthetic probe
  5' amino modifier C6
cccaaacgcatccaaagttagggtacaa

SEQ ID NO: 913 - DNA, 28 bp, Artificial Sequence
  Description of Artificial Sequence: Synthetic probe
  5' amino modifier C6
cccaaccactcgtagtctactaggagaa

SEQ ID NO: 914 - DNA, 28 bp, Artificial Sequence
  Description of Artificial Sequence: Synthetic probe
  5' amino modifier C6
cccaaactgtgttgtctcactagaggaa

SEQ ID NO: 915 - DNA, 28 bp, Artificial Sequence
  Description of Artificial Sequence: Synthetic probe
  5' amino modifier C6
cccaagtactcctactcgtacatggcaa

SEQ ID NO: 916 - DNA, 28 bp, Artificial Sequence
  Description of Artificial Sequence: Synthetic probe
  5' amino modifier C6
cccaataacacgaaagcttgtgcatcaa

SEQ ID NO: 917 - DNA, 28 bp, Artificial Sequence
  Description of Artificial Sequence: Synthetic probe
  5' amino modifier C6
cccaatttctagaactgtgcttgcacaa

SEQ ID NO: 918 - DNA, 28 bp, Artificial Sequence
  Description of Artificial Sequence: Synthetic probe
  5' amino modifier C6
cccaaggtgtacctttgaccagtgagaa

SEQ ID NO: 919 - DNA, 28 bp, Artificial Sequence
  Description of Artificial Sequence: Synthetic probe
  5' amino modifier C6
cccaagttacctcttgccatacgagaaa

SEQ ID NO: 920 - DNA, 28 bp, Artificial Sequence
  Description of Artificial Sequence: Synthetic probe
  5' amino modifier C6
cccaagaacgttctgctcatagcaaaaa

SEQ ID NO: 921 - DNA, 28 bp, Artificial Sequence
  Description of Artificial Sequence: Synthetic probe
  5' amino modifier C6
cccaaacgcttcttcattgtaacaggaa

SEQ ID NO: 922 - DNA, 28 bp, Artificial Sequence
  Description of Artificial Sequence: Synthetic probe
  5' amino modifier C6
cccaagagtctcgactcctctactagaa

SEQ ID NO: 923 - DNA, 28 bp, Artificial Sequence
  Description of Artificial Sequence: Synthetic probe
  5' amino modifier C6
cccaagagtacagaacctcactttcgaa

SEQ ID NO: 924 - DNA, 28 bp, Artificial Sequence
  Description of Artificial Sequence: Synthetic probe
  5' amino modifier C6
cccaagtactgctgacacaactaacgaa

SEQ ID NO: 925 - DNA, 28 bp, Artificial Sequence
  Description of Artificial Sequence: Synthetic probe
  5' amino modifier C6
cccaaagcctttggtagtcagacagtaa

SEQ ID NO: 926 - DNA, 28 bp, Artificial Sequence
  Description of Artificial Sequence: Synthetic probe
  5' amino modifier C6
cccaaaggctactcagaacaactttgaa

SEQ ID NO: 927 - DNA, 28 bp, Artificial Sequence
  Description of Artificial Sequence: Synthetic probe
  5' amino modifier C6
cccaagtacctcactcaagcatcaggaa

SEQ ID NO: 928 - DNA, 28 bp, Artificial Sequence
  Description of Artificial Sequence: Synthetic probe
  5' amino modifier C6
cccaaatagtctcagtgtgctagtgcaa

SEQ ID NO: 929 - DNA, 28 bp, Artificial Sequence
  Description of Artificial Sequence: Synthetic probe
  5' amino modifier C6
cccaagtccactttctgcactaagggaa

SEQ ID NO: 930 - DNA, 28 bp, Artificial Sequence
  Description of Artificial Sequence: Synthetic probe
  5' amino modifier C6
cccaacagtgcttgcaaacatcaaagaa

SEQ ID NO: 931 - DNA, 28 bp, Artificial Sequence
  Description of Artificial Sequence: Synthetic probe
  5' amino modifier C6
cccaaacttgtctctctgagtacaggaa

SEQ ID NO: 932 - DNA, 28 bp, Artificial Sequence
  Description of Artificial Sequence: Synthetic probe
  5' amino modifier C6
cccaaagttctccacaagtgtcagagaa

SEQ ID NO: 933 - DNA, 28 bp, Artificial Sequence
  Description of Artificial Sequence: Synthetic probe
  5' amino modifier C6
cccaagtcttcacactcagaacgtgaaa

SEQ ID NO: 934 - DNA, 28 bp, Artificial Sequence
  Description of Artificial Sequence: Synthetic probe
  5' amino modifier C6
cccaatccgaagttgcgtagactaaaaa

SEQ ID NO: 935 - DNA, 28 bp, Artificial Sequence
  Description of Artificial Sequence: Synthetic probe
  5' amino modifier C6
cccaagaaacatcgtacacagtctcgaa

SEQ ID NO: 936 - DNA, 28 bp, Artificial Sequence
  Description of Artificial Sequence: Synthetic probe
  5' amino modifier C6
cccaagaaccatcacctgtcagcatgaa

SEQ ID NO: 937 - DNA, 28 bp, Artificial Sequence
  Description of Artificial Sequence: Synthetic probe
  5' amino modifier C6
cccaacgacatacctaaagcatggtgaa

SEQ ID NO: 938 - DNA, 28 bp, Artificial Sequence
  Description of Artificial Sequence: Synthetic probe
  5' amino modifier C6
cccaaggtcacagcactttccactagaa

SEQ ID NO: 939 - DNA, 28 bp, Artificial Sequence
  Description of Artificial Sequence: Synthetic probe
  5' amino modifier C6
cccaacgagttacacgtttgcctaaaaa

SEQ ID NO: 940 - DNA, 28 bp, Artificial Sequence
  Description of Artificial Sequence: Synthetic probe
  5' amino modifier C6
cccaagtacgctagtctctcacatagaa

SEQ ID NO: 941 - DNA, 28 bp, Artificial Sequence
  Description of Artificial Sequence: Synthetic probe
  5' amino modifier C6
cccaaagtgtctgaccatacttaccgaa

SEQ ID NO: 942 - DNA, 28 bp, Artificial Sequence
  Description of Artificial Sequence: Synthetic probe
  5' amino modifier C6
cccaacgttccataccaaggacatagaa

SEQ ID NO: 943 - DNA, 28 bp, Artificial Sequence
  Description of Artificial Sequence: Synthetic probe
  5' amino modifier C6
cccaaggacttcgacttcctactaagaa

SEQ ID NO: 944 - DNA, 28 bp, Artificial Sequence
  Description of Artificial Sequence: Synthetic probe
  5' amino modifier C6
cccaatgacgttgtaaacctctcacgaa

SEQ ID NO: 945 - DNA, 28 bp, Artificial Sequence
  Description of Artificial Sequence: Synthetic probe
  5' amino modifier C6
cccaagcactgtgtaaacaaccttcgaa

SEQ ID NO: 946 - DNA, 28 bp, Artificial Sequence
  Description of Artificial Sequence: Synthetic probe
  5' amino modifier C6
cccaacatgtagagaaactctcgagaaa

SEQ ID NO: 947 - DNA, 28 bp, Artificial Sequence
  Description of Artificial Sequence: Synthetic probe
  5' amino modifier C6
cccaacagcttcctcatagtcttaggaa

SEQ ID NO: 948 - DNA, 28 bp, Artificial Sequence
  Description of Artificial Sequence: Synthetic probe
  5' amino modifier C6
cccaagtcctacacacagtcatacggaa

SEQ ID NO: 949 - DNA, 28 bp, Artificial Sequence
  Description of Artificial Sequence: Synthetic probe
  5' amino modifier C6
cccaagtccatacatccgaactgtgcaa

SEQ ID NO: 950 - DNA, 28 bp, Artificial Sequence
  Description of Artificial Sequence: Synthetic probe
  5' amino modifier C6
cccaagaacttccacttagcatgtgcaa

SEQ ID NO: 951 - DNA, 28 bp, Artificial Sequence
  Description of Artificial Sequence: Synthetic probe
  5' amino modifier C6
cccaaggttctacatcacgtacgcaaaa

SEQ ID NO: 952 - DNA, 28 bp, Artificial Sequence
  Description of Artificial Sequence: Synthetic probe
  5' amino modifier C6
cccaagagtgctaccttcgtacagaaaa

SEQ ID NO: 953 - DNA, 28 bp, Artificial Sequence
  Description of Artificial Sequence: Synthetic probe
  5' amino modifier C6
cccaaataagtcctgaaggaacgcataa

SEQ ID NO: 954 - DNA, 28 bp, Artificial Sequence
  Description of Artificial Sequence: Synthetic probe
  5' amino modifier C6
cccaagtgcaacgagacctttgacaaaa

SEQ ID NO: 955 - DNA, 28 bp, Artificial Sequence
  Description of Artificial Sequence: Synthetic probe
  5' amino modifier C6
cccaagcactgttgaaaccctttcgaaa

SEQ ID NO: 956 - DNA, 28 bp, Artificial Sequence
  Description of Artificial Sequence: Synthetic probe
  5' amino modifier C6
cccaaactcgtcacctttgggtaaacaa

SEQ ID NO: 957 - DNA, 28 bp, Artificial Sequence
  Description of Artificial Sequence: Synthetic probe
  5' amino modifier C6
cccaaagccttcttggtcatagacagaa

SEQ ID NO: 958 - DNA, 28 bp, Artificial Sequence
  Description of Artificial Sequence: Synthetic probe
  5' amino modifier C6
cccaacaacggtactttgttggtagcaa

SEQ ID NO: 959 - DNA, 28 bp, Artificial Sequence
  Description of Artificial Sequence: Synthetic probe
  5' amino modifier C6
cccaacattctggtgttacgaactggaa

SEQ ID NO: 960 - DNA, 28 bp, Artificial Sequence
  Description of Artificial Sequence: Synthetic probe
  5' amino modifier C6
cccaatgaaaccatccatgtcagagcaa

SEQ ID NO: 961 - DNA, 28 bp, Artificial Sequence
  Description of Artificial Sequence: Synthetic probe
  5' amino modifier C6
cccaaaactgaccattgtggtgtgcaaa